European Patent Specification EP 3 548 625 B1, published June 26, 2024. Title: COMPOSITIONS AND METHODS FOR ENHANCING GENE EXPRESSION. Applicant: SYNTHETIC GENOMICS INC. The sequence listing filed with the application follows.

SEQUENCE LISTING (52 sequences)

SEQ ID NO: 1 - DNA, 145 bp, Sindbis virus
atagtcagcatagtacatttcatctgactaatactacaacaccaccaccatgaatagaggattctttaacatgctcggccgccgccccttcccggcccccactgccatgtggaggccgcggagaaggaggcaggcggccccgatg

SEQ ID NO: 2 - DNA, 480 bp, Artificial Sequence
  Synthetic polynucleotide
gctcgaagtgtgtatggtgccatatacggctcaccaccatatacactgcaagaattactattcttgtgggcccctctcggtaaatcctagagggctttcctctcgttattgcgagattcgtcgttagataacggcaagttccctttcttactatcctattttcatcttgtggcttgacgggtcactgcctacgtcgtcgatctctatcaactacccttgcgacttaggcaaccttctccgctactggatttggagggagttttgttagggactggtccctggacttacccgacgcttgtgagcatagtcagcatagtacatttcatctgactaatactacaacaccaccaccatgaatagaggattctttaacatgctcggccgccgccccttcccggcccccactgccatgtggaggccgcggagaaggaggcaggcggccccgatgatggcaaccttctccgctactggatttggagg

SEQ ID NO: 3 - DNA, 66 bp, Artificial Sequence
  Synthetic polynucleotide
  misc_feature: 2A proteolytic cleavage site
ggaagcggagctactaacttcagcctgctgaagcaggctggagacgtggaggagaaccctggacct

SEQ ID NO: 4 - DNA, 1749 bp, Artificial Sequence
  Synthetic polynucleotide
  misc_feature: g-block for construction of rEx-DLP-rFF
cagaggcgcaggacttgatccatggcccacctacagcatgccacctgggccaagaaattgacctttggtccaatgagggcctcgaatattacaaggaagtcaacctgctgtacacacacgtccccatcaaggatggtgtaatacacagttaccctaattgtggccctgcctgtggctgggaaaagcaatccaacaaaatttcgtgcctcccgagagtggcacaaaatttgggctaccactattccccagacttaccaggattttgccccataccaaaagaactcgctgagcattggcccgtagtgtccaatgatagatacccgaattgcttgcaaattaccttacagcaagtatgtgaactcagtaaaccgtgctcagcgggctatatggttggacaatcggttttcgtgcagacgcctggtgtgacatcttactggcttactgaatgggtcgacggcaaagcgcgtgctctaccagattccttattctcgtccggtaggttcgagactaacagccgcgctttcctcgatgaagccgaggaaaagtttgccgccgctcaccctcatgcctgtttgggagaaattaataagtccaccgtgggaggatcccacttcatcttttcccaatatttaccaccattgctacccgcagacgctgttgccctggtaggtgcttcattggctgggaaagctgctaaagctgcttgcagcgttgttgatgtctatgctccatcatttgaaccttatctacaccctgagacactgagtcgcgtgtacaagattatgatcgatttcaagccgtgtaggcttatggtgtggagaaacgcgaccttttatgtccaagagggtgttgatgcagttacatcagcactagcagctgtgtccaaactcatcaaagtgccggccaatgagcctgtttcattccatgtggcatcagggtacagaaccaacgcgctggtagcgccccaggctaaaatttcaattggagcctacgccgccgagtgggcactgtcaactgaaccgccacctgctggttatgcgatcgtgcggcgatatattgtaaagaggctcctcagctcaacagaagtgttcttgtgccgcaggggtgttgtgtcttccacctcagtgcagaccatttgtgcactagagggatgtaaacctctgttcaacttcttacaaattggttcagtcattgggcccgtgtgactctagagtggacctgttcccatcccccgctcaactactcaggtagtggttcgcggcaacgggtacaccgcagttggtaacaagcttgtcgatagtcagcatagtacatttcatctgactaatactacaacaccaccaccatgaatagaggattctttaacatgctcggccgccgccccttcccggcccccactgccatgtggaggccgcggagaaggaggcaggcggccccgatgatggaaaatatggaaaacgacgagaacatcgtggtgggccccaagcccttctaccccatcgaggaaggcagcgccggcacccagctgcggaagtacatggaaagatacgccaagctgggcgccattgccttcaccaacgccgtgaccggcgtggactacagctacgccgagtacctggaaaagagctgctgcctgggcaaggctctgcagaactacggcctggtggtggacggccggatcgccctgtgcagcgagaactgcgaggaattcttcatccccgtgatcgccggcctgttcatcggcgtggg

SEQ ID NO: 5 - DNA, 67 bp, Artificial Sequence
  Synthetic polynucleotide
  misc_feature: primer pp1a-DLP-F
  misc_feature: RP114
gccatgtggaggccgcggagaaggaggcaggcggccccgatgatggcaaccttctccgctactggat

SEQ ID NO: 6 - DNA, 25 bp, Artificial Sequence
  Synthetic polynucleotide
  misc_feature: primer pBR322-3'SrfI-R
  misc_feature: RP115
acaatgttgcctcccacatctgcaa

SEQ ID NO: 7 - DNA, 25 bp, Artificial Sequence
  Synthetic polynucleotide
  misc_feature: primer pBR322-3'SrfI-F
  misc_feature: RP116
gggtcacaaggtagtcgccgtggtt

SEQ ID NO: 8 - DNA, 24 bp, Artificial Sequence
  Synthetic polynucleotide
  misc_feature: primer pBR322-bla-R
  misc_feature: RP117
cgtcaggtggcacttttcggggaa

SEQ ID NO: 9 - DNA, 70 bp, Artificial Sequence
  Synthetic polynucleotide
  misc_feature: primer pp1a-DLP-2A-F
agcctgctgaagcaggctggagacgtggaggagaaccctggacctatggcaaccttctccgctactggat

SEQ ID NO: 10 - DNA, 589 bp, Artificial Sequence
  Synthetic polynucleotide
  misc_feature: g-block for rEx-DLP-pp1ab-rFF
aaacaaataggggttccgcgcacatttccccgaaaagtgccacctgacgtctaagaaaccattattatcatgacattaagcatccgcctttcgttttatttgaccatgttggtatgtaatacgactcactatagctcgaagtgtgtatggtgccatatacggctcaccaccatatacactgcaagaattactattcttgtgggcccctctcggtaaatcctagagggctttcctctcgttattgcgagattcgtcgttagataacggcaagttccctttcttactatcctattttcatcttgtggcttgacgggtcactgcctacgtcgtcgatctctatcaactacccttgcgacttaggcaaccttctccgctactggatttggagggagttttgttagggactggtccctggacttacccgacgcttgtgagcatagtcagcatagtacatttcatctgactaatactacaacaccaccaccatgaatagaggattctttaacatgctcggccgccgccccttcccggcccccactgccatgtggaggccgcggagaaggaggcaggcggccccgatgatggcaac

SEQ ID NO: 11 - DNA, 655 bp, Artificial Sequence
  Synthetic polynucleotide
  misc_feature: g-block for rEx-DLP-2A-pp1ab-rFF
aaacaaataggggttccgcgcacatttccccgaaaagtgccacctgacgtctaagaaaccattattatcatgacattaagcatccgcctttcgttttatttgaccatgttggtatgtaatacgactcactatagctcgaagtgtgtatggtgccatatacggctcaccaccatatacactgcaagaattactattcttgtgggcccctctcggtaaatcctagagggctttcctctcgttattgcgagattcgtcgttagataacggcaagttccctttcttactatcctattttcatcttgtggcttgacgggtcactgcctacgtcgtcgatctctatcaactacccttgcgacttaggcaaccttctccgctactggatttggagggagttttgttagggactggtccctggacttacccgacgcttgtgagcatagtcagcatagtacatttcatctgactaatactacaacaccaccaccatgaatagaggattctttaacatgctcggccgccgccccttcccggcccccactgccatgtggaggccgcggagaaggaggcaggcggccccgatgggaagcggagctactaacttcagcctgctgaagcaggctggagacgtggaggagaaccctggacctatggcaac

SEQ ID NO: 12 - DNA, 655 bp, Artificial Sequence; identical to SEQ ID NO: 11
  Synthetic polynucleotide
  misc_feature: g-block for rEx-DLP-2A-pp1ab-DLP-rFF

SEQ ID NO: 13 - DNA, 30 bp, Artificial Sequence
  Synthetic polynucleotide
  misc_feature: primer DLP-pp1ab-screen-F
  misc_feature: RP126
cagcatcttttactttcaccagcgtttctg

SEQ ID NO: 14 - DNA, 25 bp, Artificial Sequence
  Synthetic polynucleotide
  misc_feature: primer DLP-pp1ab-screen-R
  misc_feature: RP127
ggaactggcgaagccagttttaaca

SEQ ID NO: 15 - DNA, 12529 bp, Artificial Sequence
  Synthetic polynucleotide
  misc_feature: Construct rEx-DLP-rFF
  misc_feature (1)...(18): T7 promoter
taatacgactcactatagctcgaagtgtgtatggtgccatatacggctcaccaccatatacactgcaagaattactattcttgtgggcccctctcggtaaatcctagagggctttcctctcgttattgcgagattcgtcgttagataacggcaagttccctttcttactatcctattttcatcttgtggcttgacgggtcactgccatcgtcgtcgatctctatcaactacccttgcgactatggcaaccttctccgctactggatttggagggagttttgttagggactggtccctggacttacccgacgcttgtgagcatggcgcgggattgtgctgcgaagtggacggctccaccttatgcgccgagtgttttcgcggttgcgaaggaatggagcaatgtcctggcttgttcatgggactgttaaaactggcttcgccagttccagtgggacataagttcctgattggttggtatcgagctgccaaagtcaccgggcgttacaatttccttgagctgttgcaacaccctgctttcgcccagctgcgtgtggttgatgctaggttagccattgaagaggcaagtgtgtttatttccactgaccacgcgtctgctaagcgtttccctggcgctagatttgcgctgacaccggtgtatgctaacgcttgggttgtgagcccggctgctaacagtttgatagtgaccactgaccaggaacaagatgggttctgctggttaaaacttttgccacctgaccgccgtgaggctggtttgcggttgtattacaaccattaccgcgaacaaaggaccgggtggctgtctaaaacaggacttcgcttatggcttggagacctgggtttgggcatcaatgcgagctctggagggctgaaattccacattatgaggggttcgcctcagcgagcttggcatatcacaacacgcagctgcaagctgaagagctactacgtttgtgacatctctgaagcagactggtcctgtttgcctgctggcaactacggcggctacaatccaccaggggacggagcttgcggttacaggtgcttggccttcatgaatggcgccactgttgtgtcggctggttgcagttctgacttgtggtgtgatgatgagttggcttatcgagtctttcaattgtcacccacgttcacggttaccatcccaggtgggcgagtttgtccgaatgccaagtacgcaatgatttgtgacaagcagcactggcgcgtcaaacgtgcaaagggcgtcggcctgtgtctcgatgaaagctgtttcaggggcatctgcaattgccaacgcatgagtggaccaccacctgcacccgtgtcagccgccgtgttagatcacatactggaggcggcgacgtttggcaacgttcgcgtggttacacctgaagggcagccacgccccgtaccagcgccgcgagttcgtcccagcgccaactcttctggagatgtcaaagatccggcgcccgttccgccagtaccaaaaccaaggaccaagcttgccacaccgaacccaactcaggcgcccatcccagcaccgcgcacgcgacttcaaggggcctcaacacaggagccactggcgagtgcaggagttgcttctgactcggcacctaaatggcgtgtggccaaaactgtgtacagctccgcggagcgctttcggaccgaactggtacaacgtgctcggtccgttggggacgttcttgttcaagcgctaccgctcaaaaccccagcagtgcagcggtataccatgactctgaagatgatgcgttcacgcttcagttggcactgcgacgtgtggtaccctttggctgtaatcgcttgtttgctccctatatggccatctcttgctttgctccttagctttgccattgggttgatacccagtgtgggcaataatgttgttctgacagcgcttctggtttcatcagctaattatgttgcgtcaatggaccatcaatgtgaaggtgcggcttgcttagccttgctggaagaagaacactattatagagcggtccgttggcgcccgattacaggcgcgctgtcgcttgtgctcaatttactggggcaggtaggctatgtagctcgttccacctttgatgcagcttatgttccttgcactgtgttcgatctttgcagctttgctattctgtacctctgccgcaatcgttgctggagatgcttcggacgctgtgtgcgagttgggcctgccacgcatgttttgggctccaccgggcaacgagtttccaaactggcgctcattgatttgtgtgaccacttttcaaagcccaccatcgatgttgtgggcatggcaactggttggagcggatgttacacaggaaccgccgcaatggagcgtcagtgtgcctctacggtggaccctcactcgttcgaccagaagaaggcaggagcgactgtttacctcaccccccctgtcaacagcgggtcagcgctgcagtgcctcaatgtcatgtggaagcgaccaattgggtccactgtccttggggaacaaacaggagctgttgtgacggcggtcaagagtatctctttctcacctccctgctgcgtctctaccactttgcccacccgacccggtgtgaccgttgtcgaccatgctctttacaaccggttgactgcttcaggggtcgatcccgctttattgcgtgttgggcaaggtgattttctaaaacttaatccggggttccggctgataggtggatggatttatgggatatgctattttgtgttggtggttgtgtcaacttttacctgcttacctatcaaatgtggcattggcacccgcgaccctttctgccgcagagtgttttctgtacccgtcaccaagacccaagagcactgccatgctggaatgtgtgctagcgctgaaggcatctctctggactctctggggttaactcagttacaaagttactggatcgcagccgtcactagcggattagtgatcttgttggtctgccaccgcctggccatcagcgccttggacttgttgactctagcttcccctttagtgttgcttgtgttcccttgggcatctgtggggcttttacttgcttgcagtctcgctggtgctgctgtgaaaatacagttgttggcgacgctttttgtgaatctattctttccccaagctacccttgtcactatgggatactgggcgtgcgtggcggctttggccgtttacagtttgatgggcttgcgagtgaaagtgaatgtgcccatgtgtgtgacacctgcccattttctgctgctggcgaggtcagctggacagtcaagagagcagatgctccgggtcagcgctgctgcccccaccaattcactgcttggagtggctcgtgattgttatgtcacaggcacaactcggctgtacatacccaaggaaggcgggatggtgtttgaagggctattcaggtcaccgaaggcgcgcggcaacgtcggcttcgtggctggtagcagctacggcacagggtcagtgtggaccaggaacaacgaggtcgtcgtactgacagcgtcacacgtggttggccgcgctaacatggccactctgaagatcggtgacgcaatgctgactctgactttcaaaaagaatggcgacttcgccgaggcagtgacgacacagtccgagctcccaggcaattggccacagttgcatttcgcccaaccaacaaccgggcccgcttcatggtgcactgccacaggagatgaagaaggcttgctcagtggcgaggtttgtctggcgtggactactagtggcgactctggatctgcagtggttcagggtgacgctgtggtaggggtccacaccggttcgaacacaagtggtgttgcctacgtgaccaccccaagcggaaaactccttggcgccgacaccgtgactttgtcatcactgtcaaagcatttcacaggccctttgacatcaatcccgaaggacatccctgacaacattattgccgatgttgatgctgttcctcgttctctggccatgctgattgatggcttatccaatagagagagcagcctttctggacctcagttgttgttaattgcttgttttatgtggtcttatcttaaccaacctgcttacttgccttatgtgctgggcttctttgccgctaacttcttcctgccaaaaagtgttggccgccctgtggtcactgggcttctatggttgtgctgcctcttcacaccgctttccatgcgcttgtgcttgttccatctggtctgtgctaccgtcacgggaaacgtgatatctttgtggttctacatcactgccgctggcacgtcttacctttctgagatgtggttcggaggctatcccaccatgttgtttgtgccacggttcctagtgtaccagttccccggctgggctattggcacagtactagcggtatgcagcatcaccatgctggctgctgccctcggtcacaccctgttactggatgtgttctccgcctcaggtcgctttgacaggactttcatgatgaaatacttcctggagggaggagtgaaagagagtgtcaccgcctcagtcacccgcgcttatggcaaaccaattacccaggagagtctcactgcaacattagctgccctcactgatgatgacttccaattcctctctgatgtgcttgactgtcgggccgtccgatcggcaatgaatctgcgtgccgctctcacaagttttcaagtggcgcagtatcgtaacatccttaatgcatccttgcaagtcgatcgtgacgctgctcgtagtcgcagactaatggcaaaactggctgattttgcggttgaacaagaagtaacagctggagaccgtgttgtggttatcgacggtctggaccgcatggctcacttcaaagacgatttggtgctggttcctttgaccaccaaagtagtaggcggttctaggtgcaccatttgtgacgtcgttaaggaagaagccaatgacaccccagttaagccaatgcccagcaggagacgccgcaagggcctgcctaaaggtgctcagttggagtgggaccgtcaccaggaagagaagaggaacgccggtgatgatgattttgcggtctcgaatgattatgtcaagagagtgccaaagtactgggatcccagcgacacccgaggcacgacagtgaaaatcgccggcactacctatcagaaagtggttgactattcaggcaatgtgcattacgtggagcatcaggaagatctgctagactacgtgctgggcaaggggagctatgaaggcctagatcaggacaaagtgttggacctcacaaacatgcttaaagtggaccccacggagctctcctccaaagacaaagccaaggcgcgtcagcttgctcatctgctgttggatctggctaacccagttgaggcagtgaatcagttaaactgagagcgccccacatctttcccggcgatgtggggcgtcggacctttgctgactctaaagacaagggtttcgtggctctacacagtcgcacaatgtttttagctgcccgggactttttatttaacatcaaatttgtgtgcgacgaagagttcacaaagaccccaaaagacacactgcttgggtacgtacgcgcctgccctggttactggtttattttccgtcgtacgcaccggtcgctgattgatgcatactgggacagtatggagtgcgtttacgcgcttcccaccatatctgattttgatgtgagcccaggtgacgtcgcagtgacgggcgagcgatgggattttgaatctcccggaggaggccgtgcaaaacgtctcacagctgatctggtgcacgcttttcaagggttccacggagcctcttattcctatgatgacaaggtggcagctgctgtcagtggtgacccgtatcggtcggacggcgtcttgtataacacccgttggggcaacattccatattctgtcccaaccaatgctttggaagccacagcttgctaccgtgctggatgtgaggccgttaccgacgggaccaacgtcatcgcaacaattgggcccttcccggagcaacaacccataccggacatcccaaagagcgtgcttgacaactgcgctgacatcagctgtgacgctttcatagcgcccgctgcagagacagccctgtgtggagatttagagaaatacaacctatccacgcagggttttgtgttgcctagtgttttctccatggtgcgggcgtacttaaaagaggagattggagacgctccaccactctacttgccatctactgtaccatctaaaaattcacaagccggaattaacggcgctgagtttcctacaaagtctttacagagctactgtttgattgatgacatggtgtcacagtccatgaaaagcaatctacaaaccgccaccatggcgacttgtaaacggcaatactgttccaaatacaagattaggagcattctgggcaccaacaattacattggcctaggtttgcgtgcctgcctttcgggggttacggccgcattccaaaaagctggaaaggatgggtcaccgatttatttgggcaagtcaaaattcgacccgataccagctcctgacaagtactgccttgaaacagacctggagagttgtgatcgctccaccccggctttggtgcgttggttcgctactaatcttatttttgagctagctggccagcccgagttggtgcacagctacgtgttgaattgctgtcacgatctagttgtggcgggtagtgtagcattcaccaaacgcgggggtttgtcatctggagaccctatcacttccatttccaataccatctattcattggtgctgtacacccagcacatgttgctatgtggacttgaaggctatttcccagagattgcagaaaaatatcttgatggcagcctggagctgcgggacatgttcaagtacgttcgagtgtacatctactcggacgatgtggttctaaccacacccaaccagcattacgcggccagctttgaccgctgggtcccccacctgcaggcgctgctaggtttcaaggttgacccaaagaaaactgtgaacaccagctccccttcctttttgggctgccggttcaagcaagtggacggcaagtgttatctagccagtcttcaggaccgcgttacacgctctctgttataccacattggtgcaaagaatccctcagagtactatgaagctgctgtttccatctttaaggactccattatctgctgtgatgaagactggtggacggacctccatcgacgtatcagtggcgctgcgcgtaccgacggagttgagttccccaccattgaaatgttaacatccttccgcaccaagcagtatgagagtgccgtgtgcacagtttgtggggccgcccccgtggccaagtctgcttgtggagggtggttctgtggcaattgtgtcccgtaccacgcgggtcattgtcacacaacctcgctcttcgccaactgcgggcacgacatcatgtaccgctccacttactgcacaatgtgtgagggttccccaaaacagatggtaccaaaagtgcctcacccgatcctggatcatttgctgtgccacattgattacggcagtaaagaggaactaactctggtagtggcggatggtcgaacaacatcaccgcccgggcgctacaaagtgggtcacaaggtagtcgccgtggttgcagatgtgggaggcaacattgtgtttgggtgcggtcctggatcacacatcgcagtaccacttcaggatacgctcaagggcgtggtggtgaataaagctctgaagaacgccgccgcctctgagtacgtggaaggaccccctgggagtgggaagacttttcacctggtcaaagatgtgctagccgtggtcggtagcgcgaccttggttgtgcccacccacgcgtccatgctggactgcatcaacaagctcaaacaagcgggcgccgatccatactttgtggtgcccaagtatacagttcttgactttccccggcctggcagtggaaacatcacagtgcgactgccacaggtcggaaccagtgagggagaaacctttgtggatgaggtggcctacttctcaccagtggatctggcgcgcattttaacccagggtcgagtcaagggttacggtgatttaaatcagctcgggtgcgtcggacccgcgagcgtgccacgtaacctttggctccgacattttgtcagcctggagcccttgcgagtgtgccatcgattcggcgctgctgtgtgtgatttgatcaagggcatttatccttattatgagccagctccacataccactaaagtggtgtttgtgccaaatccagactttgagaaaggtgtagtcatcaccgcctaccacaaagatcgcggtcttggtcaccgcacaattgattcaattcaaggctgtacattccctgttgtgactcttcgactgcccacaccccaatcactgacgcgcccgcgcgcagttgtggcggttactagggcgtctcaggaattatacatctacgacccctttgatcagcttagcgggttgttgaagttcaccaaggaagcagaggcgcaggacttgatccatggcccacctacagcatgccacctgggccaagaaattgacctttggtccaatgagggcctcgaatattacaaggaagtcaacctgctgtacacacacgtccccatcaaggatggtgtaatacacagttaccctaattgtggccctgcctgtggctgggaaaagcaatccaacaaaatttcgtgcctcccgagagtggcacaaaatttgggctaccactattccccagacttaccaggattttgccccataccaaaagaactcgctgagcattggcccgtagtgtccaatgatagatacccgaattgcttgcaaattaccttacagcaagtatgtgaactcagtaaaccgtgctcagcgggctatatggttggacaatcggttttcgtgcagacgcctggtgtgacatcttactggcttactgaatgggtcgacggcaaagcgcgtgctctaccagattccttattctcgtccggtaggttcgagactaacagccgcgctttcctcgatgaagccgaggaaaagtttgccgccgctcaccctcatgcctgtttgggagaaattaataagtccaccgtgggaggatcccacttcatcttttcccaatatttaccaccattgctacccgcagacgctgttgccctggtaggtgcttcattggctgggaaagctgctaaagctgcttgcagcgttgttgatgtctatgctccatcatttgaaccttatctacaccctgagacactgagtcgcgtgtacaagattatgatcgatttcaagccgtgtaggcttatggtgtggagaaacgcgaccttttatgtccaagagggtgttgatgcagttacatcagcactagcagctgtgtccaaactcatcaaagtgccggccaatgagcctgtttcattccatgtggcatcagggtacagaaccaacgcgctggtagcgccccaggctaaaatttcaattggagcctacgccgccgagtgggcactgtcaactgaaccgccacctgctggttatgcgatcgtgcggcgatatattgtaaagaggctcctcagctcaacagaagtgttcttgtgccgcaggggtgttgtgtcttccacctcagtgcagaccatttgtgcactagagggatgtaaacctctgttcaacttcttacaaattggttcagtcattgggcccgtgtgactctagagtggacctgttcccatcccccgctcaactactcaggtagtggttcgcggcaacgggtacaccgcagttggtaacaagcttgtcgatagtcagcatagtacatttcatctgactaatactacaacaccaccaccatgaatagaggattctttaacatgctcggccgccgccccttcccggcccccactgccatgtggaggccgcggagaaggaggcaggcggccccgatgatggaaaatatggaaaacgacgagaacatcgtggtgggccccaagcccttctaccccatcgaggaaggcagcgccggcacccagctgcggaagtacatggaaagatacgccaagctgggcgccattgccttcaccaacgccgtgaccggcgtggactacagctacgccgagtacctggaaaagagctgctgcctgggcaaggctctgcagaactacggcctggtggtggacggccggatcgccctgtgcagcgagaactgcgaggaattcttcatccccgtgatcgccggcctgttcatcggcgtgggcgtggctcccaccaacgagatctacaccctgcgggagctggtgcacagcctgggcatcagcaagcccaccatcgtgttcagcagcaagaagggcctggacaaagtcatcaccgtgcagaaaaccgtgaccaccatcaagaccatcgtgatcctggacagcaaggtggactaccggggctaccagtgcctggacaccttcatcaagcggaacaccccccctggcttccaggccagcagcttcaagaccgtggaggtggaccggaaagaacaggtggccctgatcatgaacagcagcggcagcaccggcctgcccaagggcgtgcagctgacccacgagaacaccgtgacccggttcagccacgccagggaccccatctacggcaaccaggtgtcccccggcaccgccgtgctgaccgtggtgcccttccaccacggcttcggcatgttcaccaccctgggctacctgatctgcggcttccgggtggtgatgctgaccaagttcgacgaggaaaccttcctgaaaaccctgcaggactacaagtgcacctacgtgattctggtgcccaccctgttcgccatcctgaacaagagcgagctgctgaacaagtacgacctgagcaacctggtggagatcgccagcggcggagcccccctgagcaaagaagtgggagaggccgtcgccaggcggttcaatctgcccggcgtgcggcagggctacggcctgaccgagacaaccagcgccatcatcatcacccccgagggcgacgacaagcctggagccagcggcaaggtggtgcccctgttcaaggccaaagtgatcgacctggacaccaagaagagcctgggccccaacagacggggcgaagtgtgcgtgaagggccccatgctgatgaagggctacgtgaacaaccccgaggccaccaaagagctgatcgacgaagagggctggctgcacaccggcgacatcggctactacgacgaagagaagcacttcttcatcgtggaccggctgaagagcctgatcaagtacaagggctatcaggtgccccctgccgagctggaaagcgtcctgctgcagcaccccagcatcttcgacgccggcgtggccggggtgccagatcctgtggccggcgagctgcctggcgccgtggtggtgctggaatccggcaagaacatgaccgagaaagaagtgatggactacgtcgccagccaggtgtccaacgccaagcggctgagaggcggcgtgagattcgtggacgaagtgccaaagggcctgaccggcaagatcgacggcagggccatccgggagatcctgaagaaacccgtggccaagatgtgattataactcgagggagccatagattcattttgtggtgacgggattttaggtgagtatctagattactttattctgtccgtcccactcttgctgttgcttactaggtatgtagcatctgggttagtgtatgttttgactgccttgttctattcctttgtattagcagcttatatttggtttgttatagttggaagagccttttctactgcttatgcttttgtgcttttggctgcttttctgttattagtaatgaggatgattgtgggtatgatgcctcgtcttcggtccattttcaaccatcgccaactggtggtagctgattttgtggacacacctagtggacctgttcccatcccccgcccaaccactcaggtagtggttcgcggcaacgggtacaccgcagttggtaacaagcttgtcgatggcgtcaagacgatcacgtccgcaggccgcctcttttcgaaacggacggcggcgacagcctacaagctacaatgacctactgcgcatgtttggtcagatgcgggtccgcaaaccgcccgcgcaacccactcaggctattattgcagagcctggagaccttaggcatgatttaaatcaacaggagcgcgccaccctttcgtcgaacgtacaacggttcttcatgattgggcatggttcactcactgcagatgccggaggactcacgtacaccgtcagttgggttcctaccaaacaaatccagcgcaaagttgcgcctccagcagggccgtaagacgtggatattctcctgtgtggcgtcatgttgaagtagttattagccacccaggaaccaaaaaaaaaaaaaaaaaaaaaaaaaaaaaaaaaaaaaaaaaaaaaaaaaaaaaaaaaaaaaaaaa

SEQ ID NO: 16 - DNA, 12608 bp, Artificial Sequence
  Synthetic polynucleotide
  misc_feature: Construct rEx-DLP-pp1ab-rFF
  misc_feature (1)...(18): T7 promoter
taatacgactcactatagctcgaagtgtgtatggtgccatatacggctcaccaccatatacactgcaagaattactattcttgtgggcccctctcggtaaatcctagagggctttcctctcgttattgcgagattcgtcgttagataacggcaagttccctttcttactatcctattttcatcttgtggcttgacgggtcactgcctacgtcgtcgatctctatcaactacccttgcgacttaggcaaccttctccgctactggatttggagggagttttgttagggactggtccctggacttacccgacgcttgtgagcatagtcagcatagtacatttcatctgactaatactacaacaccaccaccatgaatagaggattctttaacatgctcggccgccgccccttcccggcccccactgccatgtggaggccgcggagaaggaggcaggcggccccgatgatggcaaccttctccgctactggatttggagggagttttgttagggactggtccctggacttacccgacgcttgtgagcatggcgcgggattgtgctgcgaagtggacggctccaccttatgcgccgagtgttttcgcggttgcgaaggaatggagcaatgtcctggcttgttcatgggactgttaaaactggcttcgccagttccagtgggacataagttcctgattggttggtatcgagctgccaaagtcaccgggcgttacaatttccttgagctgttgcaacaccctgctttcgcccagctgcgtgtggttgatgctaggttagccattgaagaggcaagtgtgtttatttccactgaccacgcgtctgctaagcgtttccctggcgctagatttgcgctgacaccggtgtatgctaacgcttgggttgtgagcccggctgctaacagtttgatagtgaccactgaccaggaacaagatgggttctgctggttaaaacttttgccacctgaccgccgtgaggctggtttgcggttgtattacaaccattaccgcgaacaaaggaccgggtggctgtctaaaacaggacttcgcttatggcttggagacctgggtttgggcatcaatgcgagctctggagggctgaaattccacattatgaggggttcgcctcagcgagcttggcatatcacaacacgcagctgcaagctgaagagctactacgtttgtgacatctctgaagcagactggtcctgtttgcctgctggcaactacggcggctacaatccaccaggggacggagcttgcggttacaggtgcttggccttcatgaatggcgccactgttgtgtcggctggttgcagttctgacttgtggtgtgatgatgagttggcttatcgagtctttcaattgtcacccacgttcacggttaccatcccaggtgggcgagtttgtccgaatgccaagtacgcaatgatttgtgacaagcagcactggcgcgtcaaacgtgcaaagggcgtcggcctgtgtctcgatgaaagctgtttcaggggcatctgcaattgccaacgcatgagtggaccaccacctgcacccgtgtcagccgccgtgttagatcacatactggaggcggcgacgtttggcaacgttcgcgtggttacacctgaagggcagccacgccccgtaccagcgccgcgagttcgtcccagcgccaactcttctggagatgtcaaagatccggcgcccgttccgccagtaccaaaaccaaggaccaagcttgccacaccgaacccaactcaggcgcccatcccagcaccgcgcacgcgacttcaaggggcctcaacacaggagccactggcgagtgcaggagttgcttctgactcggcacctaaatggcgtgtggccaaaactgtgtacagctccgcggagcgctttcggaccgaactggtacaacgtgctcggtccgttggggacgttcttgttcaagcgctaccgctcaaaaccccagcagtgcagcggtataccatgactctgaagatgatgcgttcacgcttcagttggcactgcgacgtgtggtaccctttggctgtaatcgcttgtttgctccctatatggccatctcttgctttgctccttagctttgccattgggttgatacccagtgtgggcaataatgttgttctgacagcgcttctggtttcatcagctaattatgttgcgtcaatggaccatcaatgtgaaggtgcggcttgcttagccttgctggaagaagaacactattatagagcggtccgttggcgcccgattacaggcgcgctgtcgcttgtgctcaatttactggggcaggtaggctatgtagctcgttccacctttgatgcagcttatgttccttgcactgtgttcgatctttgcagctttgctattctgtacctctgccgcaatcgttgctggagatgcttcggacgctgtgtgcgagttgggcctgccacgcatgttttgggctccaccgggcaacgagtttccaaactggcgctcattgatttgtgtgaccacttttcaaagcccaccatcgatgttgtgggcatggcaactggttggagcggatgttacacaggaaccgccgcaatggagcgtcagtgtgcctctacggtggaccctcactcgttcgaccagaagaaggcaggagcgactgtttacctcaccccccctgtcaacagcgggtcagcgctgcagtgcctcaatgtcatgtggaagcgaccaattgggtccactgtccttggggaacaaacaggagctgttgtgacggcggtcaagagtatctctttctcacctccctgctgcgtctctaccactttgcccacccgacccggtgtgaccgttgtcgaccatgctctttacaaccggttgactgcttcaggggtcgatcccgctttattgcgtgttgggcaaggtgattttctaaaacttaatccggggttccggctgataggtggatggatttatgggatatgctattttgtgttggtggttgtgtcaacttttacctgcttacctatcaaatgtggcattggcacccgcgaccctttctgccgcagagtgttttctgtacccgtcaccaagacccaagagcactgccatgctggaatgtgtgctagcgctgaaggcatctctctggactctctggggttaactcagttacaaagttactggatcgcagccgtcactagcggattagtgatcttgttggtctgccaccgcctggccatcagcgccttggacttgttgactctagcttcccctttagtgttgcttgtgttcccttgggcatctgtggggcttttacttgcttgcagtctcgctggtgctgctgtgaaaatacagttgttggcgacgctttttgtgaatctattctttccccaagctacccttgtcactatgggatactgggcgtgcgtggcggctttggccgtttacagtttgatgggcttgcgagtgaaagtgaatgtgcccatgtgtgtgacacctgcccattttctgctgctggcgaggtcagctggacagtcaagagagcagatgctccgggtcagcgctgctgcccccaccaattcactgcttggagtggctcgtgattgttatgtcacaggcacaactcggctgtacatacccaaggaaggcgggatggtgtttgaagggctattcaggtcaccgaaggcgcgcggcaacgtcggcttcgtggctggtagcagctacggcacagggtcagtgtggaccaggaacaacgaggtcgtcgtactgacagcgtcacacgtggttggccgcgctaacatggccactctgaagatcggtgacgcaatgctgactctgactttcaaaaagaatggcgacttcgccgaggcagtgacgacacagtccgagctcccaggcaattggccacagttgcatttcgcccaaccaacaaccgggcccgcttcatggtgcactgccacaggagatgaagaaggcttgctcagtggcgaggtttgtctggcgtggactactagtggcgactctggatctgcagtggttcagggtgacgctgtggtaggggtccacaccggttcgaacacaagtggtgttgcctacgtgaccaccccaagcggaaaactccttggcgccgacaccgtgactttgtcatcactgtcaaagcatttcacaggccctttgacatcaatcccgaaggacatccctgacaacattattgccgatgttgatgctgttcctcgttctctggccatgctgattgatggcttatccaatagagagagcagcctttctggacctcagttgttgttaattgcttgttttatgtggtcttatcttaaccaacctgcttacttgccttatgtgctgggcttctttgccgctaacttcttcctgccaaaaagtgttggccgccctgtggtcactgggcttctatggttgtgctgcctcttcacaccgctttccatgcgcttgtgcttgttccatctggtctgtgctaccgtcacgggaaacgtgatatctttgtggttctacatcactgccgctggcacgtcttacctttctgagatgtggttcggaggctatcccaccatgttgtttgtgccacggttcctagtgtaccagttccccggctgggctattggcacagtactagcggtatgcagcatcaccatgctggctgctgccctcggtcacaccctgttactggatgtgttctccgcctcaggtcgctttgacaggactttcatgatgaaatacttcctggagggaggagtgaaagagagtgtcaccgcctcagtcacccgcgcttatggcaaaccaattacccaggagagtctcactgcaacattagctgccctcactgatgatgacttccaattcctctctgatgtgcttgactgtcgggccgtccgatcggcaatgaatctgcgtgccgctctcacaagttttcaagtggcgcagtatcgtaacatccttaatgcatccttgcaagtcgatcgtgacgctgctcgtagtcgcagactaatggcaaaactggctgattttgcggttgaacaagaagtaacagctggagaccgtgttgtggttatcgacggtctggaccgcatggctcacttcaaagacgatttggtgctggttcctttgaccaccaaagtagtaggcggttctaggtgcaccatttgtgacgtcgttaaggaagaagccaatgacaccccagttaagccaatgcccagcaggagacgccgcaagggcctgcctaaaggtgctcagttggagtgggaccgtcaccaggaagagaagaggaacgccggtgatgatgattttgcggtctcgaatgattatgtcaagagagtgccaaagtactgggatcccagcgacacccgaggcacgacagtgaaaatcgccggcactacctatcagaaagtggttgactattcaggcaatgtgcattacgtggagcatcaggaagatctgctagactacgtgctgggcaaggggagctatgaaggcctagatcaggacaaagtgttggacctcacaaacatgcttaaagtggaccccacggagctctcctccaaagacaaagccaaggcgcgtcagcttgctcatctgctgttggatctggctaacccagttgaggcagtgaatcagttaaactgagagcgccccacatctttcccggcgatgtggggcgtcggacctttgctgactctaaagacaagggtttcgtggctctacacagtcgcacaatgtttttagctgcccgggactttttatttaacatcaaatttgtgtgcgacgaagagttcacaaagaccccaaaagacacactgcttgggtacgtacgcgcctgccctggttactggtttattttccgtcgtacgcaccggtcgctgattgatgcatactgggacagtatggagtgcgtttacgcgcttcccaccatatctgattttgatgtgagcccaggtgacgtcgcagtgacgggcgagcgatgggattttgaatctcccggaggaggccgtgcaaaacgtctcacagctgatctggtgcacgcttttcaagggttccacggagcctcttattcctatgatgacaaggtggcagctgctgtcagtggtgacccgtatcggtcggacggcgtcttgtataacacccgttggggcaacattccatattctgtcccaaccaatgctttggaagccacagcttgctaccgtgctggatgtgaggccgttaccgacgggaccaacgtcatcgcaacaattgggcccttcccggagcaacaacccataccggacatcccaaagagcgtgcttgacaactgcgctgacatcagctgtgacgctttcatagcgcccgctgcagagacagccctgtgtggagatttagagaaatacaacctatccacgcagggttttgtgttgcctagtgttttctccatggtgcgggcgtacttaaaagaggagattggagacgctccaccactctacttgccatctactgtaccatctaaaaattcacaagccggaattaacggcgctgagtttcctacaaagtctttacagagctactgtttgattgatgacatggtgtcacagtccatgaaaagcaatctacaaaccgccaccatggcgacttgtaaacggcaatactgttccaaatacaagattaggagcattctgggcaccaacaattacattggcctaggtttgcgtgcctgcctttcgggggttacggccgcattccaaaaagctggaaaggatgggtcaccgatttatttgggcaagtcaaaattcgacccgataccagctcctgacaagtactgccttgaaacagacctggagagttgtgatcgctccaccccggctttggtgcgttggttcgctactaatcttatttttgagctagctggccagcccgagttggtgcacagctacgtgttgaattgctgtcacgatctagttgtggcgggtagtgtagcattcaccaaacgcgggggtttgtcatctggagaccctatcacttccatttccaataccatctattcattggtgctgtacacccagcacatgttgctatgtggacttgaaggctatttcccagagattgcagaaaaatatcttgatggcagcctggagctgcgggacatgttcaagtacgttcgagtgtacatctactcggacgatgtggttctaaccacacccaaccagcattacgcggccagctttgaccgctgggtcccccacctgcaggcgctgctaggtttcaaggttgacccaaagaaaactgtgaacaccagctccccttcctttttgggctgccggttcaagcaagtggacggcaagtgttatctagccagtcttcaggaccgcgttacacgctctctgttataccacattggtgcaaagaatccctcagagtactatgaagctgctgtttccatctttaaggactccattatctgctgtgatgaagactggtggacggacctccatcgacgtatcagtggcgctgcgcgtaccgacggagttgagttccccaccattgaaatgttaacatccttccgcaccaagcagtatgagagtgccgtgtgcacagtttgtggggccgcccccgtggccaagtctgcttgtggagggtggttctgtggcaattgtgtcccgtaccacgcgggtcattgtcacacaacctcgctcttcgccaactgcgggcacgacatcatgtaccgctccacttactgcacaatgtgtgagggttccccaaaacagatggtaccaaaagtgcctcacccgatcctggatcatttgctgtgccacattgattacggcagtaaagaggaactaactctggtagtggcggatggtcgaacaacatcaccgcccgggcgctacaaagtgggtcacaaggtagtcgccgtggttgcagatgtgggaggcaacattgtgtttgggtgcggtcctggatcacacatcgcagtaccacttcaggatacgctcaagggcgtggtggtgaataaagctctgaagaacgccgccgcctctgagtacgtggaaggaccccctgggagtgggaagacttttcacctggtcaaagatgtgctagccgtggtcggtagcgcgaccttggttgtgcccacccacgcgtccatgctggactgcatcaacaagctcaaacaagcgggcgccgatccatactttgtggtgcccaagtatacagttcttgactttccccggcctggcagtggaaacatcacagtgcgactgccacaggtcggaaccagtgagggagaaacctttgtggatgaggtggcctacttctcaccagtggatctggcgcgcattttaacccagggtcgagtcaagggttacggtgatttaaatcagctcgggtgcgtcggacccgcgagcgtgccacgtaacctttggctccgacattttgtcagcctggagcccttgcgagtgtgccatcgattcggcgctgctgtgtgtgatttgatcaagggcatttatccttattatgagccagctccacataccactaaagtggtgtttgtgccaaatccagactttgagaaaggtgtagtcatcaccgcctaccacaaagatcgcggtcttggtcaccgcacaattgattcaattcaaggctgtacattccctgttgtgactcttcgactgcccacaccccaatcactgacgcgcccgcgcgcagttgtggcggttactagggcgtctcaggaattatacatctacgacccctttgatcagcttagcgggttgttgaagttcaccaaggaagcagaggcgcaggacttgatccatggcccacctacagcatgccacctgggccaagaaattgacctttggtccaatgagggcctcgaatattacaaggaagtcaacctgctgtacacacacgtccccatcaaggatggtgtaatacacagttaccctaattgtggccctgcctgtggctgggaaaagcaatccaacaaaatttcgtgcctcccgagagtggcacaaaatttgggctaccactattccccagacttaccaggattttgccccataccaaaagaactcgctgagcattggcccgtagtgtccaatgatagatacccgaattgcttgcaaattaccttacagcaagtatgtgaactcagtaaaccgtgctcagcgggctatatggttggacaatcggttttcgtgcagacgcctggtgtgacatcttactggcttactgaatgggtcgacggcaaagcgcgtgctctaccagattccttattctcgtccggtaggttcgagactaacagccgcgctttcctcgatgaagccgaggaaaagtttgccgccgctcaccctcatgcctgtttgggagaaattaataagtccaccgtgggaggatcccacttcatcttttcccaatatttaccaccattgctacccgcagacgctgttgccctggtaggtgcttcattggctgggaaagctgctaaagctgcttgcagcgttgttgatgtctatgctccatcatttgaaccttatctacaccctgagacactgagtcgcgtgtacaagattatgatcgatttcaagccgtgtaggcttatggtgtggagaaacgcgaccttttatgtccaagagggtgttgatgcagttacatcagcactagcagctgtgtccaaactcatcaaagtgccggccaatgagcctgtttcattccatgtggcatcagggtacagaaccaacgcgctggtagcgccccaggctaaaatttcaattggagcctacgccgccgagtgggcactgtcaactgaaccgccacctgctggttatgcgatcgtgcggcgatatattgtaaagaggctcctcagctcaacagaagtgttcttgtgccgcaggggtgttgtgtcttccacctcagtgcagaccatttgtgcactagagggatgtaaacctctgttcaacttcttacaaattggttcagtcattgggcccgtgtgactctagagtggacctgttcccatcccccgctcaactactcaggtagtggttcgcggcaacgggtacaccgcagttggtaacaagcttgtcgatggaaaatatggaaaacgacgagaacatcgtggtgggccccaagcccttctaccccatcgaggaaggcagcgccggcacccagctgcggaagtacatggaaagatacgccaagctgggcgccattgccttcaccaacgccgtgaccggcgtggactacagctacgccgagtacctggaaaagagctgctgcctgggcaaggctctgcagaactacggcctggtggtggacggccggatcgccctgtgcagcgagaactgcgaggaattcttcatccccgtgatcgccggcctgttcatcggcgtgggcgtggctcccaccaacgagatctacaccctgcgggagctggtgcacagcctgggcatcagcaagcccaccatcgtgttcagcagcaagaagggcctggacaaagtcatcaccgtgcagaaaaccgtgaccaccatcaagaccatcgtgatcctggacagcaaggtggactaccggggctaccagtgcctggacaccttcatcaagcggaacaccccccctggcttccaggccagcagcttcaagaccgtggaggtggaccggaaagaacaggtggccctgatcatgaacagcagcggcagcaccggcctgcccaagggcgtgcagctgacccacgagaacaccgtgacccggttcagccacgccagggaccccatctacggcaaccaggtgtcccccggcaccgccgtgctgaccgtggtgcccttccaccacggcttcggcatgttcaccaccctgggctacctgatctgcggcttccgggtggtgatgctgaccaagttcgacgaggaaaccttcctgaaaaccctgcaggactacaagtgcacctacgtgattctggtgcccaccctgttcgccatcctgaacaagagcgagctgctgaacaagtacgacctgagcaacctggtggagatcgccagcggcggagcccccctgagcaaagaagtgggagaggccgtcgccaggcggttcaatctgcccggcgtgcggcagggctacggcctgaccgagacaaccagcgccatcatcatcacccccgagggcgacgacaagcctggagccagcggcaaggtggtgcccctgttcaaggccaaagtgatcgacctggacaccaagaagagcctgggccccaacagacggggcgaagtgtgcgtgaagggccccatgctgatgaagggctacgtgaacaaccccgaggccaccaaagagctgatcgacgaagagggctggctgcacaccggcgacatcggctactacgacgaagagaagcacttcttcatcgtggaccggctgaagagcctgatcaagtacaagggctatcaggtgccccctgccgagctggaaagcgtcctgctgcagcaccccagcatcttcgacgccggcgtggccggggtgccagatcctgtggccggcgagctgcctggcgccgtggtggtgctggaatccggcaagaacatgaccgagaaagaagtgatggactacgtcgccagccaggtgtccaacgccaagcggctgagaggcggcgtgagattcgtggacgaagtgccaaagggcctgaccggcaagatcgacggcagggccatccgggagatcctgaagaaacccgtggccaagatgtgattataactcgagggagccatagattcattttgtggtgacgggattttaggtgagtatctagattactttattctgtccgtcccactcttgctgttgcttactaggtatgtagcatctgggttagtgtatgttttgactgccttgttctattcctttgtattagcagcttatatttggtttgttatagttggaagagccttttctactgcttatgcttttgtgcttttggctgcttttctgttattagtaatgaggatgattgtgggtatgatgcctcgtcttcggtccattttcaaccatcgccaactggtggtagctgattttgtggacacacctagtggacctgttcccatcccccgcccaaccactcaggtagtggttcgcggcaacgggtacaccgcagttggtaacaagcttgtcgatggcgtcaagacgatcacgtccgcaggccgcctcttttcgaaacggacggcggcgacagcctacaagctacaatgacctactgcgcatgtttggtcagatgcgggtccgcaaaccgcccgcgcaacccactcaggctattattgcagagcctggagaccttaggcatgatttaaatcaacaggagcgcgccaccctttcgtcgaacgtacaacggttcttcatgattgggcatggttcactcactgcagatgccggaggactcacgtacaccgtcagttgggttcctaccaaacaaatccagcgcaaagttgcgcctccagcagggccgtaagacgtggatattctcctgtgtggcgtcatgttgaagtagttattagccacccaggaaccaaaaaaaaaaaaaaaaaaaaaaaaaaaaaaaaaaaaaaaaaaaaaaaaaaaaaaaaaaaaaaaaa

SEQ ID NO: 17 - DNA, 12674 bp, Artificial Sequence
  Synthetic polynucleotide
  misc_feature: Construct rEx-DLP-2A-pp1ab-rFF
  misc_feature (1)...(18): T7 promoter
taatacgactcactatagctcgaagtgtgtatggtgccatatacggctcaccaccatatacactgcaagaattactattcttgtgggcccctctcggtaaatcctagagggctttcctctcgttattgcgagattcgtcgttagataacggcaagttccctttcttactatcctattttcatcttgtggcttgacgggtcactgcctacgtcgtcgatctctatcaactacccttgcgacttaggcaaccttctccgctactggatttggagggagttttgttagggactggtccctggacttacccgacgcttgtgagcatagtcagcatagtacatttcatctgactaatactacaacaccaccaccatgaatagaggattctttaacatgctcggccgccgccccttcccggcccccactgccatgtggaggccgcggagaaggaggcaggcggccccgatgggaagcggagctactaacttcagcctgctgaagcaggctggagacgtggaggagaaccctggacctatggcaaccttctccgctactggatttggagggagttttgttagggactggtccctggacttacccgacgcttgtgagcatggcgcgggattgtgctgcgaagtggacggctccaccttatgcgccgagtgttttcgcggttgcgaaggaatggagcaatgtcctggcttgttcatgggactgttaaaactggcttcgccagttccagtgggacataagttcctgattggttggtatcgagctgccaaagtcaccgggcgttacaatttccttgagctgttgcaacaccctgctttcgcccagctgcgtgtggttgatgctaggttagccattgaagaggcaagtgtgtttatttccactgaccacgcgtctgctaagcgtttccctggcgctagatttgcgctgacaccggtgtatgctaacgcttgggttgtgagcccggctgctaacagtttgatagtgaccactgaccaggaacaagatgggttctgctggttaaaacttttgccacctgaccgccgtgaggctggtttgcggttgtattacaaccattaccgcgaacaaaggaccgggtggctgtctaaaacaggacttcgcttatggcttggagacctgggtttgggcatcaatgcgagctctggagggctgaaattccacattatgaggggttcgcctcagcgagcttggcatatcacaacacgcagctgcaagctgaagagctactacgtttgtgacatctctgaagcagactggtcctgtttgcctgctggcaactacggcggctacaatccaccaggggacggagcttgcggttacaggtgcttggccttcatgaatggcgccactgttgtgtcggctggttgcagttctgacttgtggtgtgatgatgagttggcttatcgagtctttcaattgtcacccacgttcacggttaccatcccaggtgggcgagtttgtccgaatgccaagtacgcaatgatttgtgacaagcagcactggcgcgtcaaacgtgcaaagggcgtcggcctgtgtctcgatgaaagctgtttcaggggcatctgcaattgccaacgcatgagtggaccaccacctgcacccgtgtcagccgccgtgttagatcacatactggaggcggcgacgtttggcaacgttcgcgtggttacacctgaagggcagccacgccccgtaccagcgccgcgagttcgtcccagcgccaactcttctggagatgtcaaagatccggcgcccgttccgccagtaccaaaaccaaggaccaagcttgccacaccgaacccaactcaggcgcccatcccagcaccgcgcacgcgacttcaaggggcctcaacacaggagccactggcgagtgcaggagttgcttctgactcggcacctaaatggcgtgtggccaaaactgtgtacagctccgcggagcgctttcggaccgaactggtacaacgtgctcggtccgttggggacgttcttgttcaagcgctaccgctcaaaaccccagcagtgcagcggtataccatgactctgaagatgatgcgttcacgcttcagttggcactgcgacgtgtggtaccctttggctgtaatcgcttgtttgctccctatatggccatctcttgctttgctccttagctttgccattgggttgatacccagtgtgggcaataatgttgttctgacagcgcttctggtttcatcagctaattatgttgcgtcaatggaccatcaatgtgaaggtgcggcttgcttagccttgctggaagaagaacactattatagagcggtccgttggcgcccgattacaggcgcgctgtcgcttgtgctcaatttactggggcaggtaggctatgtagctcgttccacctttgatgcagcttatgttccttgcactgtgttcgatctttgcagctttgctattctgtacctctgccgcaatcgttgctggagatgcttcggacgctgtgtgcgagttgggcctgccacgcatgttttgggctccaccgggcaacgagtttccaaactggcgctcattgatttgtgtgaccacttttcaaagcccaccatcgatgttgtgggcatggcaactggttggagcggatgttacacaggaaccgccgcaatggagcgtcagtgtgcctctacggtggaccctcactcgttcgaccagaagaaggcaggagcgactgtttacctcaccccccctgtcaacagcgggtcagcgctgcagtgcctcaatgtcatgtggaagcgaccaattgggtccactgtccttggggaacaaacaggagctgttgtgacggcggtcaagagtatctctttctcacctccctgctgcgtctctaccactttgcccacccgacccggtgtgaccgttgtcgaccatgctctttacaaccggttgactgcttcaggggtcgatcccgctttattgcgtgttgggcaaggtgattttctaaaacttaatccggggttccggctgataggtggatggatttatgggatatgctattttgtgttggtggttgtgtcaacttttacctgcttacctatcaaatgtggcattggcacccgcgaccctttctgccgcagagtgttttctgtacccgtcaccaagacccaagagcactgccatgctggaatgtgtgctagcgctgaaggcatctctctggactctctggggttaactcagttacaaagttactggatcgcagccgtcactagcggattagtgatcttgttggtctgccaccgcctggccatcagcgccttggacttgttgactctagcttcccctttagtgttgcttgtgttcccttgggcatctgtggggcttttacttgcttgcagtctcgctggtgctgctgtgaaaatacagttgttggcgacgctttttgtgaatctattctttccccaagctacccttgtcactatgggatactgggcgtgcgtggcggctttggccgtttacagtttgatgggcttgcgagtgaaagtgaatgtgcccatgtgtgtgacacctgcccattttctgctgctggcgaggtcagctggacagtcaagagagcagatgctccgggtcagcgctgctgcccccaccaattcactgcttggagtggctcgtgattgttatgtcacaggcacaactcggctgtacatacccaaggaaggcgggatggtgtttgaagggctattcaggtcaccgaaggcgcgcggcaacgtcggcttcgtggctggtagcagctacggcacagggtcagtgtggaccaggaacaacgaggtcgtcgtactgacagcgtcacacgtggttggccgcgctaacatggccactctgaagatcggtgacgcaatgctgactctgactttcaaaaagaatggcgacttcgccgaggcagtgacgacacagtccgagctcccaggcaattggccacagttgcatttcgcccaaccaacaaccgggcccgcttcatggtgcactgccacaggagatgaagaaggcttgctcagtggcgaggtttgtctggcgtggactactagtggcgactctggatctgcagtggttcagggtgacgctgtggtaggggtccacaccggttcgaacacaagtggtgttgcctacgtgaccaccccaagcggaaaactccttggcgccgacaccgtgactttgtcatcactgtcaaagcatttcacaggccctttgacatcaatcccgaaggacatccctgacaacattattgccgatgttgatgctgttcctcgttctctggccatgctgattgatggcttatccaatagagagagcagcctttctggacctcagttgttgttaattgcttgttttatgtggtcttatcttaaccaacctgcttacttgccttatgtgctgggcttctttgccgctaacttcttcctgccaaaaagtgttggccgccctgtggtcactgggcttctatggttgtgctgcctcttcacaccgctttccatgcgcttgtgcttgttccatctggtctgtgctaccgtcacgggaaacgtgatatctttgtggttctacatcactgccgctggcacgtcttacctttctgagatgtggttcggaggctatcccaccatgttgtttgtgccacggttcctagtgtaccagttccccggctgggctattggcacagtactagcggtatgcagcatcaccatgctggctgctgccctcggtcacaccctgttactggatgtgttctccgcctcaggtcgctttgacaggactttcatgatgaaatacttcctggagggaggagtgaaagagagtgtcaccgcctcagtcacccgcgcttatggcaaaccaattacccaggagagtctcactgcaacattagctgccctcactgatgatgacttccaattcctctctgatgtgcttgactgtcgggccgtccgatcggcaatgaatctgcgtgccgctctcacaagttttcaagtggcgcagtatcgtaacatccttaatgcatccttgcaagtcgatcgtgacgctgctcgtagtcgcagactaatggcaaaactggctgattttgcggttgaacaagaagtaacagctggagaccgtgttgtggttatcgacggtctggaccgcatggctcacttcaaagacgatttggtgctggttcctttgaccaccaaagtagtaggcggttctaggtgcaccatttgtgacgtcgttaaggaagaagccaatgacaccccagttaagccaatgcccagcaggagacgccgcaagggcctgcctaaaggtgctcagttggagtgggaccgtcaccaggaagagaagaggaacgccggtgatgatgattttgcggtctcgaatgattatgtcaagagagtgccaaagtactgggatcccagcgacacccgaggcacgacagtgaaaatcgccggcactacctatcagaaagtggttgactattcaggcaatgtgcattacgtggagcatcaggaagatctgctagactacgtgctgggcaaggggagctatgaaggcctagatcaggacaaagtgttggacctcacaaacatgcttaaagtggaccccacggagctctcctccaaagacaaagccaaggcgcgtcagcttgctcatctgctgttggatctggctaacccagttgaggcagtgaatcagttaaactgagagcgccccacatctttcccggcgatgtggggcgtcggacctttgctgactctaaagacaagggtttcgtggctctacacagtcgcacaatgtttttagctgcccgggactttttatttaacatcaaatttgtgtgcgacgaagagttcacaaagaccccaaaagacacactgcttgggtacgtacgcgcctgccctggttactggtttattttccgtcgtacgcaccggtcgctgattgatgcatactgggacagtatggagtgcgtttacgcgcttcccaccatatctgattttgatgtgagcccaggtgacgtcgcagtgacgggcgagcgatgggattttgaatctcccggaggaggccgtgcaaaacgtctcacagctgatctggtgcacgcttttcaagggttccacggagcctcttattcctatgatgacaaggtggcagctgctgtcagtggtgacccgtatcggtcggacggcgtcttgtataacacccgttggggcaacattccatattctgtcccaaccaatgctttggaagccacagcttgctaccgtgctggatgtgaggccgttaccgacgggaccaacgtcatcgcaacaattgggcccttcccggagcaacaacccataccggacatcccaaagagcgtgcttgacaactgcgctgacatcagctgtgacgctttcatagcgcccgctgcagagacagccctgtgtggagatttagagaaatacaacctatccacgcagggttttgtgttgcctagtgttttctccatggtgcgggcgtacttaaaagaggagattggagacgctccaccactctacttgccatctactgtaccatctaaaaattcacaagccggaattaacggcgctgagtttcctacaaagtctttacagagctactgtttgattgatgacatggtgtcacagtccatgaaaagcaatctacaaaccgccaccatggcgacttgtaaacggcaatactgttccaaatacaagattaggagcattctgggcaccaacaattacattggcctaggtttgcgtgcctgcctttcgggggttacggccgcattccaaaaagctggaaaggatgggtcaccgatttatttgggcaagtcaaaattcgacccgataccagctcctgacaagtactgccttgaaacagacctggagagttgtgatcgctccaccccggctttggtgcgttggttcgctactaatcttatttttgagctagctggccagcccgagttggtgcacagctacgtgttgaattgctgtcacgatctagttgtggcgggtagtgtagcattcaccaaacgcgggggtttgtcatctggagaccctatcacttccatttccaataccatctattcattggtgctgtacacccagcacatgttgctatgtggacttgaaggctatttcccagagattgcagaaaaatatcttgatggcagcctggagctgcgggacatgttcaagtacgttcgagtgtacatctactcggacgatgtggttctaaccacacccaaccagcattacgcggccagctttgaccgctgggtcccccacctgcaggcgctgctaggtttcaaggttgacccaaagaaaactgtgaacaccagctccccttcctttttgggctgccggttcaagcaagtggacggcaagtgttatctagccagtcttcaggaccgcgttacacgctctctgttataccacattggtgcaaagaatccctcagagtactatgaagctgctgtttccatctttaaggactccattatctgctgtgatgaagactggtggacggacctccatcgacgtatcagtggcgctgcgcgtaccgacggagttgagttccccaccattgaaatgttaacatccttccgcaccaagcagtatgagagtgccgtgtgcacagtttgtggggccgcccccgtggccaagtctgcttgtggagggtggttctgtggcaattgtgtcccgtaccacgcgggtcattgtcacacaacctcgctcttcgccaactgcgggcacgacatcatgtaccgctccacttactgcacaatgtgtgagggttccccaaaacagatggtaccaaaagtgcctcacccgatcctggatcatttgctgtgccacattgattacggcagtaaagaggaactaactctggtagtggcggatggtcgaacaacatcaccgcccgggcgctacaaagtgggtcacaaggtagtcgccgtggttgcagatgtgggaggcaacattgtgtttgggtgcggtcctggatcacacatcgcagtaccacttcaggatacgctcaagggcgtggtggtgaataaagctctgaagaacgccgccgcctctgagtacgtggaaggaccccctgggagtgggaagacttttcacctggtcaaagatgtgctagccgtggtcggtagcgcgaccttggttgtgcccacccacgcgtccatgctggactgcatcaacaagctcaaacaagcgggcgccgatccatactttgtggtgcccaagtatacagttcttgactttccccggcctggcagtggaaacatcacagtgcgactgccacaggtcggaaccagtgagggagaaacctttgtggatgaggtggcctacttctcaccagtggatctggcgcgcattttaacccagggtcgagtcaagggttacggtgatttaaatcagctcgggtgcgtcggacccgcgagcgtgccacgtaacctttggctccgacattttgtcagcctggagcccttgcgagtgtgccatcgattcggcgctgctgtgtgtgatttgatcaagggcatttatccttattatgagccagctccacataccactaaagtggtgtttgtgccaaatccagactttgagaaaggtgtagtcatcaccgcctaccacaaagatcgcggtcttggtcaccgcacaattgattcaattcaaggctgtacattccctgttgtgactcttcgactgcccacaccccaatcactgacgcgcccgcgcgcagttgtggcggttactagggcgtctcaggaattatacatctacgacccctttgatcagcttagcgggttgttgaagttcaccaaggaagcagaggcgcaggacttgatccatggcccacctacagcatgccacctgggccaagaaattgacctttggtccaatgagggcctcgaatattacaaggaagtcaacctgctgtacacacacgtccccatcaaggatggtgtaatacacagttaccctaattgtggccctgcctgtggctgggaaaagcaatccaacaaaatttcgtgcctcccgagagtggcacaaaatttgggctaccactattccccagacttaccaggattttgccccataccaaaagaactcgctgagcattggcccgtagtgtccaatgatagatacccgaattgcttgcaaattaccttacagcaagtatgtgaactcagtaaaccgtgctcagcgggctatatggttggacaatcggttttcgtgcagacgcctggtgtgacatcttactggcttactgaatgggtcgacggcaaagcgcgtgctctaccagattccttattctcgtccggtaggttcgagactaacagccgcgctttcctcgatgaagccgaggaaaagtttgccgccgctcaccctcatgcctgtttgggagaaattaataagtccaccgtgggaggatcccacttcatcttttcccaatatttaccaccattgctacccgcagacgctgttgccctggtaggtgcttcattggctgggaaagctgctaaagctgcttgcagcgttgttgatgtctatgctccatcatttgaaccttatctacaccctgagacactgagtcgcgtgtacaagattatgatcgatttcaagccgtgtaggcttatggtgtggagaaacgcgaccttttatgtccaagagggtgttgatgcagttacatcagcactagcagctgtgtccaaactcatcaaagtgccggccaatgagcctgtttcattccatgtggcatcagggtacagaaccaacgcgctggtagcgccccaggctaaaatttcaattggagcctacgccgccgagtgggcactgtcaactgaaccgccacctgctggttatgcgatcgtgcggcgatatattgtaaagaggctcctcagctcaacagaagtgttcttgtgccgcaggggtgttgtgtcttccacctcagtgcagaccatttgtgcactagagggatgtaaacctctgttcaacttcttacaaattggttcagtcattgggcccgtgtgactctagagtggacctgttcccatcccccgctcaactactcaggtagtggttcgcggcaacgggtacaccgcagttggtaacaagcttgtcgatggaaaatatggaaaacgacgagaacatcgtggtgggccccaagcccttctaccccatcgaggaaggcagcgccggcacccagctgcggaagtacatggaaagatacgccaagctgggcgccattgccttcaccaacgccgtgaccggcgtggactacagctacgccgagtacctggaaaagagctgctgcctgggcaaggctctgcagaactacggcctggtggtggacggccggatcgccctgtgcagcgagaactgcgaggaattcttcatccccgtgatcgccggcctgttcatcggcgtgggcgtggctcccaccaacgagatctacaccctgcgggagctggtgcacagcctgggcatcagcaagcccaccatcgtgttcagcagcaagaagggcctggacaaagtcatcaccgtgcagaaaaccgtgaccaccatcaagaccatcgtgatcctggacagcaaggtggactaccggggctaccagtgcctggacaccttcatcaagcggaacaccccccctggcttccaggccagcagcttcaagaccgtggaggtggaccggaaagaacaggtggccctgatcatgaacagcagcggcagcaccggcctgcccaagggcgtgcagctgacccacgagaacaccgtgacccggttcagccacgccagggaccccatctacggcaaccaggtgtcccccggcaccgccgtgctgaccgtggtgcccttccaccacggcttcggcatgttcaccaccctgggctacctgatctgcggcttccgggtggtgatgctgaccaagttcgacgaggaaaccttcctgaaaaccctgcaggactacaagtgcacctacgtgattctggtgcccaccctgttcgccatcctgaacaagagcgagctgctgaacaagtacgacctgagcaacctggtggagatcgccagcggcggagcccccctgagcaaagaagtgggagaggccgtcgccaggcggttcaatctgcccggcgtgcggcagggctacggcctgaccgagacaaccagcgccatcatcatcacccccgagggcgacgacaagcctggagccagcggcaaggtggtgcccctgttcaaggccaaagtgatcgacctggacaccaagaagagcctgggccccaacagacggggcgaagtgtgcgtgaagggccccatgctgatgaagggctacgtgaacaaccccgaggccaccaaagagctgatcgacgaagagggctggctgcacaccggcgacatcggctactacgacgaagagaagcacttcttcatcgtggaccggctgaagagcctgatcaagtacaagggctatcaggtgccccctgccgagctggaaagcgtcctgctgcagcaccccagcatcttcgacgccggcgtggccggggtgccagatcctgtggccggcgagctgcctggcgccgtggtggtgctggaatccggcaagaacatgaccgagaaagaagtgatggactacgtcgccagccaggtgtccaacgccaagcggctgagaggcggcgtgagattcgtggacgaagtgccaaagggcctgaccggcaagatcgacggcagggccatccgggagatcctgaagaaacccgtggccaagatgtgattataactcgagggagccatagattcattttgtggtgacgggattttaggtgagtatctagattactttattctgtccgtcccactcttgctgttgcttactaggtatgtagcatctgggttagtgtatgttttgactgccttgttctattcctttgtattagcagcttatatttggtttgttatagttggaagagccttttctactgcttatgcttttgtgcttttggctgcttttctgttattagtaatgaggatgattgtgggtatgatgcctcgtcttcggtccattttcaaccatcgccaactggtggtagctgattttgtggacacacctagtggacctgttcccatcccccgcccaaccactcaggtagtggttcgcggcaacgggtacaccgcagttggtaacaagcttgtcgatggcgtcaagacgatcacgtccgcaggccgcctcttttcgaaacggacggcggcgacagcctacaagctacaatgacctactgcgcatgtttggtcagatgcgggtccgcaaaccgcccgcgcaacccactcaggctattattgcagagcctggagaccttaggcatgatttaaatcaacaggagcgcgccaccctttcgtcgaacgtacaacggttcttcatgattgggcatggttcactcactgcagatgccggaggactcacgtacaccgtcagttgggttcctaccaaacaaatccagcgcaaagttgcgcctccagcagggccgtaagacgtggatattctcctgtgtggcgtcatgttgaagtagttattagccacccaggaaccaaaaaaaaaaaaaaaaaaaaaaaaaaaaaaaaaaaaaaaaaaaaaaaaaaaaaaaaaaaaaaaaa

SEQ ID NO: 18 - DNA, 12819 bp, Artificial Sequence
  Synthetic polynucleotide
  misc_feature: Construct rEx-DLP-2A-pp1ab-DLP-rFF
  misc_feature (1)...(18): T7 promoter
taatacgactcactatagctcgaagtgtgtatggtgccatatacggctcaccaccatatacactgcaagaattactattcttgtgggcccctctcggtaaatcctagagggctttcctctcgttattgcgagattcgtcgttagataacggcaagttccctttcttactatcctattttcatcttgtggcttgacgggtcactgcctacgtcgtcgatctctatcaactacccttgcgacttaggcaaccttctccgctactggatttggagggagttttgttagggactggtccctggacttacccgacgcttgtgagcatagtcagcatagtacatttcatctgactaatactacaacaccaccaccatgaatagaggattctttaacatgctcggccgccgccccttcccggcccccactgccatgtggaggccgcggagaaggaggcaggcggccccgatgggaagcggagctactaacttcagcctgctgaagcaggctggagacgtggaggagaaccctggacctatggcaaccttctccgctactggatttggagggagttttgttagggactggtccctggacttacccgacgcttgtgagcatggcgcgggattgtgctgcgaagtggacggctccaccttatgcgccgagtgttttcgcggttgcgaaggaatggagcaatgtcctggcttgttcatgggactgttaaaactggcttcgccagttccagtgggacataagttcctgattggttggtatcgagctgccaaagtcaccgggcgttacaatttccttgagctgttgcaacaccctgctttcgcccagctgcgtgtggttgatgctaggttagccattgaagaggcaagtgtgtttatttccactgaccacgcgtctgctaagcgtttccctggcgctagatttgcgctgacaccggtgtatgctaacgcttgggttgtgagcccggctgctaacagtttgatagtgaccactgaccaggaacaagatgggttctgctggttaaaacttttgccacctgaccgccgtgaggctggtttgcggttgtattacaaccattaccgcgaacaaaggaccgggtggctgtctaaaacaggacttcgcttatggcttggagacctgggtttgggcatcaatgcgagctctggagggctgaaattccacattatgaggggttcgcctcagcgagcttggcatatcacaacacgcagctgcaagctgaagagctactacgtttgtgacatctctgaagcagactggtcctgtttgcctgctggcaactacggcggctacaatccaccaggggacggagcttgcggttacaggtgcttggccttcatgaatggcgccactgttgtgtcggctggttgcagttctgacttgtggtgtgatgatgagttggcttatcgagtctttcaattgtcacccacgttcacggttaccatcccaggtgggcgagtttgtccgaatgccaagtacgcaatgatttgtgacaagcagcactggcgcgtcaaacgtgcaaagggcgtcggcctgtgtctcgatgaaagctgtttcaggggcatctgcaattgccaacgcatgagtggaccaccacctgcacccgtgtcagccgccgtgttagatcacatactggaggcggcgacgtttggcaacgttcgcgtggttacacctgaagggcagccacgccccgtaccagcgccgcgagttcgtcccagcgccaactcttctggagatgtcaaagatccggcgcccgttccgccagtaccaaaaccaaggaccaagcttgccacaccgaacccaactcaggcgcccatcccagcaccgcgcacgcgacttcaaggggcctcaacacaggagccactggcgagtgcaggagttgcttctgactcggcacctaaatggcgtgtggccaaaactgtgtacagctccgcggagcgctttcggaccgaactggtacaacgtgctcggtccgttggggacgttcttgttcaagcgctaccgctcaaaaccccagcagtgcagcggtataccatgactctgaagatgatgcgttcacgcttcagttggcactgcgacgtgtggtaccctttggctgtaatcgcttgtttgctccctatatggccatctcttgctttgctccttagctttgccattgggttgatacccagtgtgggcaataatgttgttctgacagcgcttctggtttcatcagctaattatgttgcgtcaatggaccatcaatgtgaaggtgcggcttgcttagccttgctggaagaagaacactattatagagcggtccgttggcgcccgattacaggcgcgctgtcgcttgtgctcaatttactggggcaggtaggctatgtagctcgttccacctttgatgcagcttatgttccttgcactgtgttcgatctttgcagctttgctattctgtacctctgccgcaatcgttgctggagatgcttcggacgctgtgtgcgagttgggcctgccacgcatgttttgggctccaccgggcaacgagtttccaaactggcgctcattgatttgtgtgaccacttttcaaagcccaccatcgatgttgtgggcatggcaactggttggagcggatgttacacaggaaccgccgcaatggagcgtcagtgtgcctctacggtggaccctcactcgttcgaccagaagaaggcaggagcgactgtttacctcaccccccctgtcaacagcgggtcagcgctgcagtgcctcaatgtcatgtggaagcgaccaattgggtccactgtccttggggaacaaacaggagctgttgtgacggcggtcaagagtatctctttctcacctccctgctgcgtctctaccactttgcccacccgacccggtgtgaccgttgtcgaccatgctctttacaaccggttgactgcttcaggggtcgatcccgctttattgcgtgttgggcaaggtgattttctaaaacttaatccggggttccggctgataggtggatggatttatgggatatgctattttgtgttggtggttgtgtcaacttttacctgcttacctatcaaatgtggcattggcacccgcgaccctttctgccgcagagtgttttctgtacccgtcaccaagacccaagagcactgccatgctggaatgtgtgctagcgctgaaggcatctctctggactctctggggttaactcagttacaaagttactggatcgcagccgtcactagcggattagtgatcttgttggtctgccaccgcctggccatcagcgccttggacttgttgactctagcttcccctttagtgttgcttgtgttcccttgggcatctgtggggcttttacttgcttgcagtctcgctggtgctgctgtgaaaatacagttgttggcgacgctttttgtgaatctattctttccccaagctacccttgtcactatgggatactgggcgtgcgtggcggctttggccgtttacagtttgatgggcttgcgagtgaaagtgaatgtgcccatgtgtgtgacacctgcccattttctgctgctggcgaggtcagctggacagtcaagagagcagatgctccgggtcagcgctgctgcccccaccaattcactgcttggagtggctcgtgattgttatgtcacaggcacaactcggctgtacatacccaaggaaggcgggatggtgtttgaagggctattcaggtcaccgaaggcgcgcggcaacgtcggcttcgtggctggtagcagctacggcacagggtcagtgtggaccaggaacaacgaggtcgtcgtactgacagcgtcacacgtggttggccgcgctaacatggccactctgaagatcggtgacgcaatgctgactctgactttcaaaaagaatggcgacttcgccgaggcagtgacgacacagtccgagctcccaggcaattggccacagttgcatttcgcccaaccaacaaccgggcccgcttcatggtgcactgccacaggagatgaagaaggcttgctcagtggcgaggtttgtctggcgtggactactagtggcgactctggatctgcagtggttcagggtgacgctgtggtaggggtccacaccggttcgaacacaagtggtgttgcctacgtgaccaccccaagcggaaaactccttggcgccgacaccgtgactttgtcatcactgtcaaagcatttcacaggccctttgacatcaatcccgaaggacatccctgacaacattattgccgatgttgatgctgttcctcgttctctggccatgctgattgatggcttatccaatagagagagcagcctttctggacctcagttgttgttaattgcttgttttatgtggtcttatcttaaccaacctgcttacttgccttatgtgctgggcttctttgccgctaacttcttcctgccaaaaagtgttggccgccctgtggtcactgggcttctatggttgtgctgcctcttcacaccgctttccatgcgcttgtgcttgttccatctggtctgtgctaccgtcacgggaaacgtgatatctttgtggttctacatcactgccgctggcacgtcttacctttctgagatgtggttcggaggctatcccaccatgttgtttgtgccacggttcctagtgtaccagttccccggctgggctattggcacagtactagcggtatgcagcatcaccatgctggctgctgccctcggtcacaccctgttactggatgtgttctccgcctcaggtcgctttgacaggactttcatgatgaaatacttcctggagggaggagtgaaagagagtgtcaccgcctcagtcacccgcgcttatggcaaaccaattacccaggagagtctcactgcaacattagctgccctcactgatgatgacttccaattcctctctgatgtgcttgactgtcgggccgtccgatcggcaatgaatctgcgtgccgctctcacaagttttcaagtggcgcagtatcgtaacatccttaatgcatccttgcaagtcgatcgtgacgctgctcgtagtcgcagactaatggcaaaactggctgattttgcggttgaacaagaagtaacagctggagaccgtgttgtggttatcgacggtctggaccgcatggctcacttcaaagacgatttggtgctggttcctttgaccaccaaagtagtaggcggttctaggtgcaccatttgtgacgtcgttaaggaagaagccaatgacaccccagttaagccaatgcccagcaggagacgccgcaagggcctgcctaaaggtgctcagttggagtgggaccgtcaccaggaagagaagaggaacgccggtgatgatgattttgcggtctcgaatgattatgtcaagagagtgccaaagtactgggatcccagcgacacccgaggcacgacagtgaaaatcgccggcactacctatcagaaagtggttgactattcaggcaatgtgcattacgtggagcatcaggaagatctgctagactacgtgctgggcaaggggagctatgaaggcctagatcaggacaaagtgttggacctcacaaacatgcttaaagtggaccccacggagctctcctccaaagacaaagccaaggcgcgtcagcttgctcatctgctgttggatctggctaacccagttgaggcagtgaatcagttaaactgagagcgccccacatctttcccggcgatgtggggcgtcggacctttgctgactctaaagacaagggtttcgtggctctacacagtcgcacaatgtttttagctgcccgggactttttatttaacatcaaatttgtgtgcgacgaagagttcacaaagaccccaaaagacacactgcttgggtacgtacgcgcctgccctggttactggtttattttccgtcgtacgcaccggtcgctgattgatgcatactgggacagtatggagtgcgtttacgcgcttcccaccatatctgattttgatgtgagcccaggtgacgtcgcagtgacgggcgagcgatgggattttgaatctcccggaggaggccgtgcaaaacgtctcacagctgatctggtgcacgcttttcaagggttccacggagcctcttattcctatgatgacaaggtggcagctgctgtcagtggtgacccgtatcggtcggacggcgtcttgtataacacccgttggggcaacattccatattctgtcccaaccaatgctttggaagccacagcttgctaccgtgctggatgtgaggccgttaccgacgggaccaacgtcatcgcaacaattgggcccttcccggagcaacaacccataccggacatcccaaagagcgtgcttgacaactgcgctgacatcagctgtgacgctttcatagcgcccgctgcagagacagccctgtgtggagatttagagaaatacaacctatccacgcagggttttgtgttgcctagtgttttctccatggtgcgggcgtacttaaaagaggagattggagacgctccaccactctacttgccatctactgtaccatctaaaaattcacaagccggaattaacggcgctgagtttcctacaaagtctttacagagctactgtttgattgatgacatggtgtcacagtccatgaaaagcaatctacaaaccgccaccatggcgacttgtaaacggcaatactgttccaaatacaagattaggagcattctgggcaccaacaattacattggcctaggtttgcgtgcctgcctttcgggggttacggccgcattccaaaaagctggaaaggatgggtcaccgatttatttgggcaagtcaaaattcgacccgataccagctcctgacaagtactgccttgaaacagacctggagagttgtgatcgctccaccccggctttggtgcgttggttcgctactaatcttatttttgagctagctggccagcccgagttggtgcacagctacgtgttgaattgctgtcacgatctagttgtggcgggtagtgtagcattcaccaaacgcgggggtttgtcatctggagaccctatcacttccatttccaataccatctattcattggtgctgtacacccagcacatgttgctatgtggacttgaaggctatttcccagagattgcagaaaaatatcttgatggcagcctggagctgcgggacatgttcaagtacgttcgagtgtacatctactcggacgatgtggttctaaccacacccaaccagcattacgcggccagctttgaccgctgggtcccccacctgcaggcgctgctaggtttcaaggttgacccaaagaaaactgtgaacaccagctccccttcctttttgggctgccggttcaagcaagtggacggcaagtgttatctagccagtcttcaggaccgcgttacacgctctctgttataccacattggtgcaaagaatccctcagagtactatgaagctgctgtttccatctttaaggactccattatctgctgtgatgaagactggtggacggacctccatcgacgtatcagtggcgctgcgcgtaccgacggagttgagttccccaccattgaaatgttaacatccttccgcaccaagcagtatgagagtgccgtgtgcacagtttgtggggccgcccccgtggccaagtctgcttgtggagggtggttctgtggcaattgtgtcccgtaccacgcgggtcattgtcacacaacctcgctcttcgccaactgcgggcacgacatcatgtaccgctccacttactgcacaatgtgtgagggttccccaaaacagatggtaccaaaagtgcctcacccgatcctggatcatttgctgtgccacattgattacggcagtaaagaggaactaactctggtagtggcggatggtcgaacaacatcaccgcccgggcgctacaaagtgggtcacaaggtagtcgccgtggttgcagatgtgggaggcaacattgtgtttgggtgcggtcctggatcacacatcgcagtaccacttcaggatacgctcaagggcgtggtggtgaataaagctctgaagaacgccgccgcctctgagtacgtggaaggaccccctgggagtgggaagacttttcacctggtcaaagatgtgctagccgtggtcggtagcgcgaccttggttgtgcccacccacgcgtccatgctggactgcatcaacaagctcaaacaagcgggcgccgatccatactttgtggtgcccaagtatacagttcttgactttccccggcctggcagtggaaacatcacagtgcgactgccacaggtcggaaccagtgagggagaaacctttgtggatgaggtggcctacttctcaccagtggatctggcgcgcattttaacccagggtcgagtcaagggttacggtgatttaaatcagctcgggtgcgtcggacccgcgagcgtgccacgtaacctttggctccgacattttgtcagcctggagcccttgcgagtgtgccatcgattcggcgctgctgtgtgtgatttgatcaagggcatttatccttattatgagccagctccacataccactaaagtggtgtttgtgccaaatccagactttgagaaaggtgtagtcatcaccgcctaccacaaagatcgcggtcttggtcaccgcacaattgattcaattcaaggctgtacattccctgttgtgactcttcgactgcccacaccccaatcactgacgcgcccgcgcgcagttgtggcggttactagggcgtctcaggaattatacatctacgacccctttgatcagcttagcgggttgttgaagttcaccaaggaagcagaggcgcaggacttgatccatggcccacctacagcatgccacctgggccaagaaattgacctttggtccaatgagggcctcgaatattacaaggaagtcaacctgctgtacacacacgtccccatcaaggatggtgtaatacacagttaccctaattgtggccctgcctgtggctgggaaaagcaatccaacaaaatttcgtgcctcccgagagtggcacaaaatttgggctaccactattccccagacttaccaggattttgccccataccaaaagaactcgctgagcattggcccgtagtgtccaatgatagatacccgaattgcttgcaaattaccttacagcaagtatgtgaactcagtaaaccgtgctcagcgggctatatggttggacaatcggttttcgtgcagacgcctggtgtgacatcttactggcttactgaatgggtcgacggcaaagcgcgtgctctaccagattccttattctcgtccggtaggttcgagactaacagccgcgctttcctcgatgaagccgaggaaaagtttgccgccgctcaccctcatgcctgtttgggagaaattaataagtccaccgtgggaggatcccacttcatcttttcccaatatttaccaccattgctacccgcagacgctgttgccctggtaggtgcttcattggctgggaaagctgctaaagctgcttgcagcgttgttgatgtctatgctccatcatttgaaccttatctacaccctgagacactgagtcgcgtgtacaagattatgatcgatttcaagccgtgtaggcttatggtgtggagaaacgcgaccttttatgtccaagagggtgttgatgcagttacatcagcactagcagctgtgtccaaactcatcaaagtgccggccaatgagcctgtttcattccatgtggcatcagggtacagaaccaacgcgctggtagcgccccaggctaaaatttcaattggagcctacgccgccgagtgggcactgtcaactgaaccgccacctgctggttatgcgatcgtgcggcgatatattgtaaagaggctcctcagctcaacagaagtgttcttgtgccgcaggggtgttgtgtcttccacctcagtgcagaccatttgtgcactagagggatgtaaacctctgttcaacttcttacaaattggttcagtcattgggcccgtgtgactctagagtggacctgttcccatcccccgctcaactactcaggtagtggttcgcggcaacgggtacaccgcagttggtaacaagcttgtcgatagtcagcatagtacatttcatctgactaatactacaacaccaccaccatgaatagaggattctttaacatgctcggccgccgccccttcccggcccccactgccatgtggaggccgcggagaaggaggcaggcggccccgatgatggaaaatatggaaaacgacgagaacatcgtggtgggccccaagcccttctaccccatcgaggaaggcagcgccggcacccagctgcggaagtacatggaaagatacgccaagctgggcgccattgccttcaccaacgccgtgaccggcgtggactacagctacgccgagtacctggaaaagagctgctgcctgggcaaggctctgcagaactacggcctggtggtggacggccggatcgccctgtgcagcgagaactgcgaggaattcttcatccccgtgatcgccggcctgttcatcggcgtgggcgtggctcccaccaacgagatctacaccctgcgggagctggtgcacagcctgggcatcagcaagcccaccatcgtgttcagcagcaagaagggcctggacaaagtcatcaccgtgcagaaaaccgtgaccaccatcaagaccatcgtgatcctggacagcaaggtggactaccggggctaccagtgcctggacaccttcatcaagcggaacaccccccctggcttccaggccagcagcttcaagaccgtggaggtggaccggaaagaacaggtggccctgatcatgaacagcagcggcagcaccggcctgcccaagggcgtgcagctgacccacgagaacaccgtgacccggttcagccacgccagggaccccatctacggcaaccaggtgtcccccggcaccgccgtgctgaccgtggtgcccttccaccacggcttcggcatgttcaccaccctgggctacctgatctgcggcttccgggtggtgatgctgaccaagttcgacgaggaaaccttcctgaaaaccctgcaggactacaagtgcacctacgtgattctggtgcccaccctgttcgccatcctgaacaagagcgagctgctgaacaagtacgacctgagcaacctggtggagatcgccagcggcggagcccccctgagcaaagaagtgggagaggccgtcgccaggcggttcaatctgcccggcgtgcggcagggctacggcctgaccgagacaaccagcgccatcatcatcacccccgagggcgacgacaagcctggagccagcggcaaggtggtgcccctgttcaaggccaaagtgatcgacctggacaccaagaagagcctgggccccaacagacggggcgaagtgtgcgtgaagggccccatgctgatgaagggctacgtgaacaaccccgaggccaccaaagagctgatcgacgaagagggctggctgcacaccggcgacatcggctactacgacgaagagaagcacttcttcatcgtggaccggctgaagagcctgatcaagtacaagggctatcaggtgccccctgccgagctggaaagcgtcctgctgcagcaccccagcatcttcgacgccggcgtggccggggtgccagatcctgtggccggcgagctgcctggcgccgtggtggtgctggaatccggcaagaacatgaccgagaaagaagtgatggactacgtcgccagccaggtgtccaacgccaagcggctgagaggcggcgtgagattcgtggacgaagtgccaaagggcctgaccggcaagatcgacggcagggccatccgggagatcctgaagaaacccgtggccaagatgtgattataactcgagggagccatagattcattttgtggtgacgggattttaggtgagtatctagattactttattctgtccgtcccactcttgctgttgcttactaggtatgtagcatctgggttagtgtatgttttgactgccttgttctattcctttgtattagcagcttatatttggtttgttatagttggaagagccttttctactgcttatgcttttgtgcttttggctgcttttctgttattagtaatgaggatgattgtgggtatgatgcctcgtcttcggtccattttcaaccatcgccaactggtggtagctgattttgtggacacacctagtggacctgttcccatcccccgcccaaccactcaggtagtggttcgcggcaacgggtacaccgcagttggtaacaagcttgtcgatggcgtcaagacgatcacgtccgcaggccgcctcttttcgaaacggacggcggcgacagcctacaagctacaatgacctactgcgcatgtttggtcagatgcgggtccgcaaaccgcccgcgcaacccactcaggctattattgcagagcctggagaccttaggcatgatttaaatcaacaggagcgcgccaccctttcgtcgaacgtacaacggttcttcatgattgggcatggttcactcactgcagatgccggaggactcacgtacaccgtcagttgggttcctaccaaacaaatccagcgcaaagttgcgcctccagcagggccgtaagacgtggatattctcctgtgtggcgtcatgttgaagtagttattagccacccaggaaccaaaaaaaaaaaaaaaaaaaaaaaaaaaaaaaaaaaaaaaaaaaaaaaaaaaaaaaaaaaaaaaaa

SEQ ID NO: 19 - DNA, 464 bp, Artificial Sequence
  Synthetic polynucleotide
  misc_feature: Construct Alpha-R-DLP-2A-nsp-rFF
gataggcggcgcatgagagaagcccagaccaattacctacccaaataggagaaagttcacgttgacatcgaggaagacagcccattcctcagagctttgcagcggagcttcccgcagtttgaggtagaagccaagcaggtcactgataatgaccatgctaatgccagagcgttttcgcatctggcttcaaaactgatcgaaacggaggtggacccatccgacacgatccttgacattggaatagtcagcatagtacatttcatctgactaatactacaacaccaccaccatgaatagaggattctttaacatgctcggccgccgccccttcccggcccccactgccatgtggaggccgcggagaaggaggcaggcggccccgggaagcggagctactaacttcagcctgctgaagcaggctggagacgtggaggagaaccctggacctatggagaaagttcacg

SEQ ID NO: 20 - DNA, 80 bp, Artificial Sequence
  Synthetic polynucleotide
  misc_feature: primer DLP-rFF-F
  misc_feature: RP112
cctgaatggactacgacatagtctagtccgccaagatatcgcaccatagtcagcatagtacatttcatctgactaatact

SEQ ID NO: 21 - DNA, 60 bp, Artificial Sequence
  Synthetic polynucleotide
  misc_feature: primer DLP-rFF-R
  misc_feature: RP113
gcagcttgccaattgctgctgtatcgatcaattaatcacatcttggccacgggtttcttc

SEQ ID NO: 22 - DNA, 67 bp, Artificial Sequence
  Synthetic polynucleotide
  misc_feature: primer 5'Alpha-P2A-F
  misc_feature: RP124
gaagcaggctggagacgtggaggagaaccctggacctgagaaagttcacgttgacatcgaggaagac

SEQ ID NO: 23 - DNA, 30 bp, Artificial Sequence
  Synthetic polynucleotide
  misc_feature: primer 5'ScaI-R
  misc_feature: RP125
caccagtcacagaaaagcatcttacggatg

SEQ ID NO: 24 - DNA, 1014 bp, Artificial Sequence
  Synthetic polynucleotide
  misc_feature: g-block for Alpha-R-DLP-2A-nsp-rFF
tgtcatgccatccgtaagatgcttttctgtgactggtgagtactcaaccaagtcattctgagaatagtgtatgcggcgaccgagttgctcttgcccggcgtcaacacgggataataccgcgccacatagcagaactttaaaagtgctcatcattggaaaacgttcttcggggcgaaaactctcaaggatcttaccgctgttgagatccagttcgatgtaacccactcgtgcacccaactgatcttcagcatcttttactttcaccagcgtttctgggtgagcaaaaacaggaaggcaaaatgccgcaaaaaagggaataagggcgacacggaaatgttgaatactcatactcttcctttttcaatattattgaagcatttatcagggttattgtctcatgagcggatacatatttgaatgtatttagaaaaataaacaaataggggttccgcgcacatttccccgaaaagtgccacctgacgtctaagaaaccattattatcatgacattaagcatccgcctttcgttttatttgaccatgttggtatgtaatacgactcactatagataggcggcgcatgagagaagcccagaccaattacctacccaaataggagaaagttcacgttgacatcgaggaagacagcccattcctcagagctttgcagcggagcttcccgcagtttgaggtagaagccaagcaggtcactgataatgaccatgctaatgccagagcgttttcgcatctggcttcaaaactgatcgaaacggaggtggacccatccgacacgatccttgacattggaatagtcagcatagtacatttcatctgactaatactacaacaccaccaccatgaatagaggattctttaacatgctcggccgccgccccttcccggcccccactgccatgtggaggccgcggagaaggaggcaggcggccccgggaagcggagctactaacttcagcctgctgaagcaggctggagacgtggaggagaaccctggacct

SEQ ID NO: 25 - DNA, 1014 bp, Artificial Sequence; identical to SEQ ID NO: 24
  Synthetic polynucleotide
  misc_feature: g-block for Alpha-R-DLP-2A-nsp-DLP-rFF

SEQ ID NO: 26 - DNA, 9476 bp, Artificial Sequence
  Synthetic polynucleotide
  misc_feature: construct Alpha-R-rFF
  misc_feature (1)...(18): T7 promoter
taatacgactcactatagataggcggcgcatgagagaagcccagaccaattacctacccaaaatggagaaagttcacgttgacatcgaggaagacagcccattcctcagagctttgcagcggagcttcccgcagtttgaggtagaagccaagcaggtcactgataatgaccatgctaatgccagagcgttttcgcatctggcttcaaaactgatcgaaacggaggtggacccatccgacacgatccttgacattggaagtgcgcccgcccgcagaatgtattctaagcacaagtatcattgtatctgtccgatgagatgtgcggaagatccggacagattgtataagtatgcaactaagctgaagaaaaactgtaaggaaataactgataaggaattggacaagaaaatgaaggagctcgccgccgtcatgagcgaccctgacctggaaactgagactatgtgcctccacgacgacgagtcgtgtcgctacgaagggcaagtcgctgtttaccaggatgtatacgcggttgacggaccgacaagtctctatcaccaagccaataagggagttagagtcgcctactggataggctttgacaccaccccttttatgtttaagaacttggctggagcatatccatcatactctaccaactgggccgacgaaaccgtgttaacggctcgtaacataggcctatgcagctctgacgttatggagcggtcacgtagagggatgtccattcttagaaagaagtatttgaaaccatccaacaatgttctattctctgttggctcgaccatctaccacgagaagagggacttactgaggagctggcacctgccgtctgtatttcacttacgtggcaagcaaaattacacatgtcggtgtgagactatagttagttgcgacgggtacgtcgttaaaagaatagctatcagtccaggcctgtatgggaagccttcaggctatgctgctacgatgcaccgcgagggattcttgtgctgcaaagtgacagacacattgaacggggagagggtctcttttcccgtgtgcacgtatgtgccagctacattgtgtgaccaaatgactggcatactggcaacagatgtcagtgcggacgacgcgcaaaaactgctggttgggctcaaccagcgtatagtcgtcaacggtcgcacccagagaaacaccaataccatgaaaaattaccttttgcccgtagtggcccaggcatttgctaggtgggcaaaggaatataaggaagatcaagaagatgaaaggccactaggactacgagatagacagttagtcatggggtgttgttgggcttttagaaggcacaagataacatctatttataagcgcccggatacccaaaccatcatcaaagtgaacagcgatttccactcattcgtgctgcccaggataggcagtaacacattggagatcgggctgagaacaagaatcaggaaaatgttagaggagcacaaggagccgtcacctctcattaccgccgaggacgtacaagaagctaagtgcgcagccgatgaggctaaggaggtgcgtgaagccgaggagttgcgcgcagctctaccacctttggcagctgatgttgaggagcccactctggaagccgatgtcgacttgatgttacaagaggctggggccggctcagtggagacacctcgtggcttgataaaggttaccagctacgatggcgaggacaagatcggctcttacgctgtgctttctccgcaggctgtactcaagagtgaaaaattatcttgcatccaccctctcgctgaacaagtcatagtgataacacactctggccgaaaagggcgttatgccgtggaaccataccatggtaaagtagtggtgccagagggacatgcaatacccgtccaggactttcaagctctgagtgaaagtgccaccattgtgtacaacgaacgtgagttcgtaaacaggtacctgcaccatattgccacacatggaggagcgctgaacactgatgaagaatattacaaaactgtcaagcccagcgagcacgacggcgaatacctgtacgacatcgacaggaaacagtgcgtcaagaaagaactagtcactgggctagggctcacaggcgagctggtggatcctcccttccatgaattcgcctacgagagtctgagaacacgaccagccgctccttaccaagtaccaaccataggggtgtatggcgtgccaggatcaggcaagtctggcatcattaaaagcgcagtcaccaaaaaagatctagtggtgagcgccaagaaagaaaactgtgcagaaattataagggacgtcaagaaaatgaaagggctggacgtcaatgccagaactgtggactcagtgctcttgaatggatgcaaacaccccgtagagaccctgtatattgacgaagcttttgcttgtcatgcaggtactctcagagcgctcatagccattataagacctaaaaaggcagtgctctgcggggatcccaaacagtgcggtttttttaacatgatgtgcctgaaagtgcattttaaccacgagatttgcacacaagtcttccacaaaagcatctctcgccgttgcactaaatctgtgacttcggtcgtctcaaccttgttttacgacaaaaaaatgagaacgacgaatccgaaagagactaagattgtgattgacactaccggcagtaccaaacctaagcaggacgatctcattctcacttgtttcagagggtgggtgaagcagttgcaaatagattacaaaggcaacgaaataatgacggcagctgcctctcaagggctgacccgtaaaggtgtgtatgccgttcggtacaaggtgaatgaaaatcctctgtacgcacccacctctgaacatgtgaacgtcctactgacccgcacggaggaccgcatcgtgtggaaaacactagccggcgacccatggataaaaacactgactgccaagtaccctgggaatttcactgccacgatagaggagtggcaagcagagcatgatgccatcatgaggcacatcttggagagaccggaccctaccgacgtcttccagaataaggcaaacgtgtgttgggccaaggctttagtgccggtgctgaagaccgctggcatagacatgaccactgaacaatggaacactgtggattattttgaaacggacaaagctcactcagcagagatagtattgaaccaactatgcgtgaggttctttggactcgatctggactccggtctattttctgcacccactgttccgttatccattaggaataatcactgggataactccccgtcgcctaacatgtacgggctgaataaagaagtggtccgtcagctctctcgcaggtacccacaactgcctcgggcagttgccactggaagagtctatgacatgaacactggtacactgcgcaattatgatccgcgcataaacctagtacctgtaaacagaagactgcctcatgctttagtcctccaccataatgaacacccacagagtgacttttcttcattcgtcagcaaattgaagggcagaactgtcctggtggtcggggaaaagttgtccgtcccaggcaaaatggttgactggttgtcagaccggcctgaggctaccttcagagctcggctggatttaggcatcccaggtgatgtgcccaaatatgacataatatttgttaatgtgaggaccccatataaataccatcactatcagcagtgtgaagaccatgccattaagcttagcatgttgaccaagaaagcttgtctgcatctgaatcccggcggaacctgtgtcagcataggttatggttacgctgacagggccagcgaaagcatcattggtgctatagcgcggcagttcaagttttcccgggtatgcaaaccgaaatcctcacttgaagagacggaagttctgtttgtattcattgggtacgatcgcaaggcccgtacgcacaatccttacaagctttcatcaaccttgaccaacatttatacaggttccagactccacgaagccggatgtgcaccctcatatcatgtggtgcgaggggatattgccacggccaccgaaggagtgattataaatgctgctaacagcaaaggacaacctggcggaggggtgtgcggagcgctgtataagaaattcccggaaagcttcgatttacagccgatcgaagtaggaaaagcgcgactggtcaaaggtgcagctaaacatatcattcatgccgtaggaccaaacttcaacaaagtttcggaggttgaaggtgacaaacagttggcagaggcttatgagtccatcgctaagattgtcaacgataacaattacaagtcagtagcgattccactgttgtccaccggcatcttttccgggaacaaagatcgactaacccaatcattgaaccatttgctgacagctttagacaccactgatgcagatgtagccatatactgcagggacaagaaatgggaaatgactctcaaggaagcagtggctaggagagaagcagtggaggagatatgcatatccgacgactcttcagtgacagaacctgatgcagagctggtgagggtgcatccgaagagttctttggctggaaggaagggctacagcacaagcgatggcaaaactttctcatatttggaagggaccaagtttcaccaggcggccaaggatatagcagaaattaatgccatgtggcccgttgcaacggaggccaatgagcaggtatgcatgtatatcctcggagaaagcatgagcagtattaggtcgaaatgccccgtcgaagagtcggaagcctccacaccacctagcacgctgccttgcttgtgcatccatgccatgactccagaaagagtacagcgcctaaaagcctcacgtccagaacaaattactgtgtgctcatcctttccattgccgaagtatagaatcactggtgtgcagaagatccaatgctcccagcctatattgttctcaccgaaagtgcctgcgtatattcatccaaggaagtatctcgtggaaacaccaccggtagacgagactccggagccatcggcagagaaccaatccacagaggggacacctgaacaaccaccacttataaccgaggatgagaccaggactagaacgcctgagccgatcatcatcgaagaggaagaagaggatagcataagtttgctgtcagatggcccgacccaccaggtgctgcaagtcgaggcagacattcacgggccgccctctgtatctagctcatcctggtccattcctcatgcatccgactttgatgtggacagtttatccatacttgacaccctggagggagctagcgtgaccagcggggcaacgtcagccgagactaactcttacttcgcaaagagtatggagtttctggcgcgaccggtgcctgcgcctcgaacagtattcaggaaccctccacatcccgctccgcgcacaagaacaccgtcacttgcacccagcagggcctgctcgagaaccagcctagtttccaccccgccaggcgtgaatagggtgatcactagagaggagctcgaggcgcttaccccgtcacgcactcctagcaggtcggtctcgagaaccagcctggtctccaacccgccaggcgtaaatagggtgattacaagagaggagtttgaggcgttcgtagcacaacaacaatgacggtttgatgcgggtgcatacatcttttcctccgacaccggtcaagggcatttacaacaaaaatcagtaaggcaaacggtgctatccgaagtggtgttggagaggaccgaattggagatttcgtatgccccgcgcctcgaccaagaaaaagaagaattactacgcaagaaattacagttaaatcccacacctgctaacagaagcagataccagtccaggaaggtggagaacatgaaagccataacagctagacgtattctgcaaggcctagggcattatttgaaggcagaaggaaaagtggagtgctaccgaaccctgcatcctgttcctttgtattcatctagtgtgaaccgtgccttttcaagccccaaggtcgcagtggaagcctgtaacgccatgttgaaagagaactttccgactgtggcttcttactgtattattccagagtacgatgcctatttggacatggttgacggagcttcatgctgcttagacactgccagtttttgccctgcaaagctgcgcagctttccaaagaaacactcctatttggaacccacaatacgatcggcagtgccttcagcgatccagaacacgctccagaacgtcctggcagctgccacaaaaagaaattgcaatgtcacgcaaatgagagaattgcccgtattggattcggcggcctttaatgtggaatgcttcaagaaatatgcgtgtaataatgaatattgggaaacgtttaaagaaaaccccatcaggcttactgaagaaaacgtggtaaattacattaccaaattaaaaggaccaaaagctgctgctctttttgcgaagacacataatttgaatatgttgcaggacataccaatggacaggtttgtaatggacttaaagagagacgtgaaagtgactccaggaacaaaacatactgaagaacggcccaaggtacaggtgatccaggctgccgatccgctagcaacagcgtatctgtgcggaatccaccgagagctggttaggagattaaatgcggtcctgcttccgaacattcatacactgtttgatatgtcggctgaagactttgacgctattatagccgagcacttccagcctggggattgtgttctggaaactgacatcgcgtcgtttgataaaagtgaggacgacgccatggctctgaccgcgttaatgattctggaagacttaggtgtggacgcagagctgttgacgctgattgaggcggctttcggcgaaatttcatcaatacatttgcccactaaaactaaatttaaattcggagccatgatgaaatctggaatgttcctcacactgtttgtgaacacagtcattaacattgtaatcgcaagcagagtgttgagagaacggctaaccggatcaccatgtgcagcattcattggagatgacaatatcgtgaaaggagtcaaatcggacaaattaatggcagacaggtgcgccacctggttgaatatggaagtcaagattatagatgctgtggtgggcgagaaagcgccttatttctgtggagggtttattttgtgtgactccgtgaccggcacagcgtgccgtgtggcagaccccctaaaaaggctgtttaagcttggcaaacctctggcagcagacgatgaacatgatgatgacaggagaagggcattgcatgaagagtcaacacgctggaaccgagtgggtattctttcagagctgtgcaaggcagtagaatcaaggtatgaaaccgtaggaacttccatcatagttatggccatgactactctagctagcagtgttaaatcattcagctacctgagaggggcccctataactctctacggctaacctgaatggactacgacatagtctagtccgccaagatatcgcaccatggaaaatatggaaaacgacgagaacatcgtggtgggccccaagcccttctaccccatcgaggaaggcagcgccggcacccagctgcggaagtacatggaaagatacgccaagctgggcgccattgccttcaccaacgccgtgaccggcgtggactacagctacgccgagtacctggaaaagagctgctgcctgggcaaggctctgcagaactacggcctggtggtggacggccggatcgccctgtgcagcgagaactgcgaggaattcttcatccccgtgatcgccggcctgttcatcggcgtgggcgtggctcccaccaacgagatctacaccctgcgggagctggtgcacagcctgggcatcagcaagcccaccatcgtgttcagcagcaagaagggcctggacaaagtcatcaccgtgcagaaaaccgtgaccaccatcaagaccatcgtgatcctggacagcaaggtggactaccggggctaccagtgcctggacaccttcatcaagcggaacaccccccctggcttccaggccagcagcttcaagaccgtggaggtggaccggaaagaacaggtggccctgatcatgaacagcagcggcagcaccggcctgcccaagggcgtgcagctgacccacgagaacaccgtgacccggttcagccacgccagggaccccatctacggcaaccaggtgtcccccggcaccgccgtgctgaccgtggtgcccttccaccacggcttcggcatgttcaccaccctgggctacctgatctgcggcttccgggtggtgatgctgaccaagttcgacgaggaaaccttcctgaaaaccctgcaggactacaagtgcacctacgtgattctggtgcccaccctgttcgccatcctgaacaagagcgagctgctgaacaagtacgacctgagcaacctggtggagatcgccagcggcggagcccccctgagcaaagaagtgggagaggccgtcgccaggcggttcaatctgcccggcgtgcggcagggctacggcctgaccgagacaaccagcgccatcatcatcacccccgagggcgacgacaagcctggagccagcggcaaggtggtgcccctgttcaaggccaaagtgatcgacctggacaccaagaagagcctgggccccaacagacggggcgaagtgtgcgtgaagggccccatgctgatgaagggctacgtgaacaaccccgaggccaccaaagagctgatcgacgaagagggctggctgcacaccggcgacatcggctactacgacgaagagaagcacttcttcatcgtggaccggctgaagagcctgatcaagtacaagggctatcaggtgccccctgccgagctggaaagcgtcctgctgcagcaccccagcatcttcgacgccggcgtggccggggtgccagatcctgtggccggcgagctgcctggcgccgtggtggtgctggaatccggcaagaacatgaccgagaaagaagtgatggactacgtcgccagccaggtgtccaacgccaagcggctgagaggcggcgtgagattcgtggacgaagtgccaaagggcctgaccggcaagatcgacggcagggccatccgggagatcctgaagaaacccgtggccaagatgtgattaattgatcgatacagcagcaattggcaagctgcttacatagaaggcgcgccgtttaaacggccggccttaattaagtaacgatacagcagcaattggcaagctgcttacatagaactcgcggcgattggcatgccgctttaaaatttttattttatttttcttttcttttccgaatcggattttgtttttaatatttcaaaaaaaaaaaaaaaaaaaaaaaaaaaaaaaaaaaaaaaa

SEQ ID NO: 27 - DNA, 9621 bp, Artificial Sequence
  Synthetic polynucleotide
  misc_feature: construct Alpha-R-DLP-rFF
  misc_feature (1)...(18): T7 promoter
taatacgactcactatagataggcggcgcatgagagaagcccagaccaattacctacccaaaatggagaaagttcacgttgacatcgaggaagacagcccattcctcagagctttgcagcggagcttcccgcagtttgaggtagaagccaagcaggtcactgataatgaccatgctaatgccagagcgttttcgcatctggcttcaaaactgatcgaaacggaggtggacccatccgacacgatccttgacattggaagtgcgcccgcccgcagaatgtattctaagcacaagtatcattgtatctgtccgatgagatgtgcggaagatccggacagattgtataagtatgcaactaagctgaagaaaaactgtaaggaaataactgataaggaattggacaagaaaatgaaggagctcgccgccgtcatgagcgaccctgacctggaaactgagactatgtgcctccacgacgacgagtcgtgtcgctacgaagggcaagtcgctgtttaccaggatgtatacgcggttgacggaccgacaagtctctatcaccaagccaataagggagttagagtcgcctactggataggctttgacaccaccccttttatgtttaagaacttggctggagcatatccatcatactctaccaactgggccgacgaaaccgtgttaacggctcgtaacataggcctatgcagctctgacgttatggagcggtcacgtagagggatgtccattcttagaaagaagtatttgaaaccatccaacaatgttctattctctgttggctcgaccatctaccacgagaagagggacttactgaggagctggcacctgccgtctgtatttcacttacgtggcaagcaaaattacacatgtcggtgtgagactatagttagttgcgacgggtacgtcgttaaaagaatagctatcagtccaggcctgtatgggaagccttcaggctatgctgctacgatgcaccgcgagggattcttgtgctgcaaagtgacagacacattgaacggggagagggtctcttttcccgtgtgcacgtatgtgccagctacattgtgtgaccaaatgactggcatactggcaacagatgtcagtgcggacgacgcgcaaaaactgctggttgggctcaaccagcgtatagtcgtcaacggtcgcacccagagaaacaccaataccatgaaaaattaccttttgcccgtagtggcccaggcatttgctaggtgggcaaaggaatataaggaagatcaagaagatgaaaggccactaggactacgagatagacagttagtcatggggtgttgttgggcttttagaaggcacaagataacatctatttataagcgcccggatacccaaaccatcatcaaagtgaacagcgatttccactcattcgtgctgcccaggataggcagtaacacattggagatcgggctgagaacaagaatcaggaaaatgttagaggagcacaaggagccgtcacctctcattaccgccgaggacgtacaagaagctaagtgcgcagccgatgaggctaaggaggtgcgtgaagccgaggagttgcgcgcagctctaccacctttggcagctgatgttgaggagcccactctggaagccgatgtcgacttgatgttacaagaggctggggccggctcagtggagacacctcgtggcttgataaaggttaccagctacgatggcgaggacaagatcggctcttacgctgtgctttctccgcaggctgtactcaagagtgaaaaattatcttgcatccaccctctcgctgaacaagtcatagtgataacacactctggccgaaaagggcgttatgccgtggaaccataccatggtaaagtagtggtgccagagggacatgcaatacccgtccaggactttcaagctctgagtgaaagtgccaccattgtgtacaacgaacgtgagttcgtaaacaggtacctgcaccatattgccacacatggaggagcgctgaacactgatgaagaatattacaaaactgtcaagcccagcgagcacgacggcgaatacctgtacgacatcgacaggaaacagtgcgtcaagaaagaactagtcactgggctagggctcacaggcgagctggtggatcctcccttccatgaattcgcctacgagagtctgagaacacgaccagccgctccttaccaagtaccaaccataggggtgtatggcgtgccaggatcaggcaagtctggcatcattaaaagcgcagtcaccaaaaaagatctagtggtgagcgccaagaaagaaaactgtgcagaaattataagggacgtcaagaaaatgaaagggctggacgtcaatgccagaactgtggactcagtgctcttgaatggatgcaaacaccccgtagagaccctgtatattgacgaagcttttgcttgtcatgcaggtactctcagagcgctcatagccattataagacctaaaaaggcagtgctctgcggggatcccaaacagtgcggtttttttaacatgatgtgcctgaaagtgcattttaaccacgagatttgcacacaagtcttccacaaaagcatctctcgccgttgcactaaatctgtgacttcggtcgtctcaaccttgttttacgacaaaaaaatgagaacgacgaatccgaaagagactaagattgtgattgacactaccggcagtaccaaacctaagcaggacgatctcattctcacttgtttcagagggtgggtgaagcagttgcaaatagattacaaaggcaacgaaataatgacggcagctgcctctcaagggctgacccgtaaaggtgtgtatgccgttcggtacaaggtgaatgaaaatcctctgtacgcacccacctctgaacatgtgaacgtcctactgacccgcacggaggaccgcatcgtgtggaaaacactagccggcgacccatggataaaaacactgactgccaagtaccctgggaatttcactgccacgatagaggagtggcaagcagagcatgatgccatcatgaggcacatcttggagagaccggaccctaccgacgtcttccagaataaggcaaacgtgtgttgggccaaggctttagtgccggtgctgaagaccgctggcatagacatgaccactgaacaatggaacactgtggattattttgaaacggacaaagctcactcagcagagatagtattgaaccaactatgcgtgaggttctttggactcgatctggactccggtctattttctgcacccactgttccgttatccattaggaataatcactgggataactccccgtcgcctaacatgtacgggctgaataaagaagtggtccgtcagctctctcgcaggtacccacaactgcctcgggcagttgccactggaagagtctatgacatgaacactggtacactgcgcaattatgatccgcgcataaacctagtacctgtaaacagaagactgcctcatgctttagtcctccaccataatgaacacccacagagtgacttttcttcattcgtcagcaaattgaagggcagaactgtcctggtggtcggggaaaagttgtccgtcccaggcaaaatggttgactggttgtcagaccggcctgaggctaccttcagagctcggctggatttaggcatcccaggtgatgtgcccaaatatgacataatatttgttaatgtgaggaccccatataaataccatcactatcagcagtgtgaagaccatgccattaagcttagcatgttgaccaagaaagcttgtctgcatctgaatcccggcggaacctgtgtcagcataggttatggttacgctgacagggccagcgaaagcatcattggtgctatagcgcggcagttcaagttttcccgggtatgcaaaccgaaatcctcacttgaagagacggaagttctgtttgtattcattgggtacgatcgcaaggcccgtacgcacaatccttacaagctttcatcaaccttgaccaacatttatacaggttccagactccacgaagccggatgtgcaccctcatatcatgtggtgcgaggggatattgccacggccaccgaaggagtgattataaatgctgctaacagcaaaggacaacctggcggaggggtgtgcggagcgctgtataagaaattcccggaaagcttcgatttacagccgatcgaagtaggaaaagcgcgactggtcaaaggtgcagctaaacatatcattcatgccgtaggaccaaacttcaacaaagtttcggaggttgaaggtgacaaacagttggcagaggcttatgagtccatcgctaagattgtcaacgataacaattacaagtcagtagcgattccactgttgtccaccggcatcttttccgggaacaaagatcgactaacccaatcattgaaccatttgctgacagctttagacaccactgatgcagatgtagccatatactgcagggacaagaaatgggaaatgactctcaaggaagcagtggctaggagagaagcagtggaggagatatgcatatccgacgactcttcagtgacagaacctgatgcagagctggtgagggtgcatccgaagagttctttggctggaaggaagggctacagcacaagcgatggcaaaactttctcatatttggaagggaccaagtttcaccaggcggccaaggatatagcagaaattaatgccatgtggcccgttgcaacggaggccaatgagcaggtatgcatgtatatcctcggagaaagcatgagcagtattaggtcgaaatgccccgtcgaagagtcggaagcctccacaccacctagcacgctgccttgcttgtgcatccatgccatgactccagaaagagtacagcgcctaaaagcctcacgtccagaacaaattactgtgtgctcatcctttccattgccgaagtatagaatcactggtgtgcagaagatccaatgctcccagcctatattgttctcaccgaaagtgcctgcgtatattcatccaaggaagtatctcgtggaaacaccaccggtagacgagactccggagccatcggcagagaaccaatccacagaggggacacctgaacaaccaccacttataaccgaggatgagaccaggactagaacgcctgagccgatcatcatcgaagaggaagaagaggatagcataagtttgctgtcagatggcccgacccaccaggtgctgcaagtcgaggcagacattcacgggccgccctctgtatctagctcatcctggtccattcctcatgcatccgactttgatgtggacagtttatccatacttgacaccctggagggagctagcgtgaccagcggggcaacgtcagccgagactaactcttacttcgcaaagagtatggagtttctggcgcgaccggtgcctgcgcctcgaacagtattcaggaaccctccacatcccgctccgcgcacaagaacaccgtcacttgcacccagcagggcctgctcgagaaccagcctagtttccaccccgccaggcgtgaatagggtgatcactagagaggagctcgaggcgcttaccccgtcacgcactcctagcaggtcggtctcgagaaccagcctggtctccaacccgccaggcgtaaatagggtgattacaagagaggagtttgaggcgttcgtagcacaacaacaatgacggtttgatgcgggtgcatacatcttttcctccgacaccggtcaagggcatttacaacaaaaatcagtaaggcaaacggtgctatccgaagtggtgttggagaggaccgaattggagatttcgtatgccccgcgcctcgaccaagaaaaagaagaattactacgcaagaaattacagttaaatcccacacctgctaacagaagcagataccagtccaggaaggtggagaacatgaaagccataacagctagacgtattctgcaaggcctagggcattatttgaaggcagaaggaaaagtggagtgctaccgaaccctgcatcctgttcctttgtattcatctagtgtgaaccgtgccttttcaagccccaaggtcgcagtggaagcctgtaacgccatgttgaaagagaactttccgactgtggcttcttactgtattattccagagtacgatgcctatttggacatggttgacggagcttcatgctgcttagacactgccagtttttgccctgcaaagctgcgcagctttccaaagaaacactcctatttggaacccacaatacgatcggcagtgccttcagcgatccagaacacgctccagaacgtcctggcagctgccacaaaaagaaattgcaatgtcacgcaaatgagagaattgcccgtattggattcggcggcctttaatgtggaatgcttcaagaaatatgcgtgtaataatgaatattgggaaacgtttaaagaaaaccccatcaggcttactgaagaaaacgtggtaaattacattaccaaattaaaaggaccaaaagctgctgctctttttgcgaagacacataatttgaatatgttgcaggacataccaatggacaggtttgtaatggacttaaagagagacgtgaaagtgactccaggaacaaaacatactgaagaacggcccaaggtacaggtgatccaggctgccgatccgctagcaacagcgtatctgtgcggaatccaccgagagctggttaggagattaaatgcggtcctgcttccgaacattcatacactgtttgatatgtcggctgaagactttgacgctattatagccgagcacttccagcctggggattgtgttctggaaactgacatcgcgtcgtttgataaaagtgaggacgacgccatggctctgaccgcgttaatgattctggaagacttaggtgtggacgcagagctgttgacgctgattgaggcggctttcggcgaaatttcatcaatacatttgcccactaaaactaaatttaaattcggagccatgatgaaatctggaatgttcctcacactgtttgtgaacacagtcattaacattgtaatcgcaagcagagtgttgagagaacggctaaccggatcaccatgtgcagcattcattggagatgacaatatcgtgaaaggagtcaaatcggacaaattaatggcagacaggtgcgccacctggttgaatatggaagtcaagattatagatgctgtggtgggcgagaaagcgccttatttctgtggagggtttattttgtgtgactccgtgaccggcacagcgtgccgtgtggcagaccccctaaaaaggctgtttaagcttggcaaacctctggcagcagacgatgaacatgatgatgacaggagaagggcattgcatgaagagtcaacacgctggaaccgagtgggtattctttcagagctgtgcaaggcagtagaatcaaggtatgaaaccgtaggaacttccatcatagttatggccatgactactctagctagcagtgttaaatcattcagctacctgagaggggcccctataactctctacggctaacctgaatggactacgacatagtctagtccgccaagatatcgcaccatagtcagcatagtacatttcatctgactaatactacaacaccaccaccatgaatagaggattctttaacatgctcggccgccgccccttcccggcccccactgccatgtggaggccgcggagaaggaggcaggcggccccgatgatggaaaatatggaaaacgacgagaacatcgtggtgggccccaagcccttctaccccatcgaggaaggcagcgccggcacccagctgcggaagtacatggaaagatacgccaagctgggcgccattgccttcaccaacgccgtgaccggcgtggactacagctacgccgagtacctggaaaagagctgctgcctgggcaaggctctgcagaactacggcctggtggtggacggccggatcgccctgtgcagcgagaactgcgaggaattcttcatccccgtgatcgccggcctgttcatcggcgtgggcgtggctcccaccaacgagatctacaccctgcgggagctggtgcacagcctgggcatcagcaagcccaccatcgtgttcagcagcaagaagggcctggacaaagtcatcaccgtgcagaaaaccgtgaccaccatcaagaccatcgtgatcctggacagcaaggtggactaccggggctaccagtgcctggacaccttcatcaagcggaacaccccccctggcttccaggccagcagcttcaagaccgtggaggtggaccggaaagaacaggtggccctgatcatgaacagcagcggcagcaccggcctgcccaagggcgtgcagctgacccacgagaacaccgtgacccggttcagccacgccagggaccccatctacggcaaccaggtgtcccccggcaccgccgtgctgaccgtggtgcccttccaccacggcttcggcatgttcaccaccctgggctacctgatctgcggcttccgggtggtgatgctgaccaagttcgacgaggaaaccttcctgaaaaccctgcaggactacaagtgcacctacgtgattctggtgcccaccctgttcgccatcctgaacaagagcgagctgctgaacaagtacgacctgagcaacctggtggagatcgccagcggcggagcccccctgagcaaagaagtgggagaggccgtcgccaggcggttcaatctgcccggcgtgcggcagggctacggcctgaccgagacaaccagcgccatcatcatcacccccgagggcgacgacaagcctggagccagcggcaaggtggtgcccctgttcaaggccaaagtgatcgacctggacaccaagaagagcctgggccccaacagacggggcgaagtgtgcgtgaagggccccatgctgatgaagggctacgtgaacaaccccgaggccaccaaagagctgatcgacgaagagggctggctgcacaccggcgacatcggctactacgacgaagagaagcacttcttcatcgtggaccggctgaagagcctgatcaagtacaagggctatcaggtgccccctgccgagctggaaagcgtcctgctgcagcaccccagcatcttcgacgccggcgtggccggggtgccagatcctgtggccggcgagctgcctggcgccgtggtggtgctggaatccggcaagaacatgaccgagaaagaagtgatggactacgtcgccagccaggtgtccaacgccaagcggctgagaggcggcgtgagattcgtggacgaagtgccaaagggcctgaccggcaagatcgacggcagggccatccgggagatcctgaagaaacccgtggccaagatgtgattaattgatcgatacagcagcaattggcaagctgcttacatagaaggcgcgccgtttaaacggccggccttaattaagtaacgatacagcagcaattggcaagctgcttacatagaactcgcggcgattggcatgccgctttaaaatttttattttatttttcttttcttttccgaatcggattttgtttttaatatttcaaaaaaaaaaaaaaaaaaaaaaaaaaaaaaaaaaaaaaaa

SEQ ID NO: 28 - DNA, 9876 bp, Artificial Sequence
  Synthetic polynucleotide
  misc_feature: construct Alpha-R-DLP-2A-nsp-rFF
  misc_feature (1)...(18): T7 promoter
taatacgactcactatagataggcggcgcatgagagaagcccagaccaattacctacccaaataggagaaagttcacgttgacatcgaggaagacagcccattcctcagagctttgcagcggagcttcccgcagtttgaggtagaagccaagcaggtcactgataatgaccatgctaatgccagagcgttttcgcatctggcttcaaaactgatcgaaacggaggtggacccatccgacacgatccttgacattggaatagtcagcatagtacatttcatctgactaatactacaacaccaccaccatgaatagaggattctttaacatgctcggccgccgccccttcccggcccccactgccatgtggaggccgcggagaaggaggcaggcggccccgggaagcggagctactaacttcagcctgctgaagcaggctggagacgtggaggagaaccctggacctgagaaagttcacgttgacatcgaggaagacagcccattcctcagagctttgcagcggagcttcccgcagtttgaggtagaagccaagcaggtcactgataatgaccatgctaatgccagagcgttttcgcatctggcttcaaaactgatcgaaacggaggtggacccatccgacacgatccttgacattggaagtgcgcccgcccgcagaatgtattctaagcacaagtatcattgtatctgtccgatgagatgtgcggaagatccggacagattgtataagtatgcaactaagctgaagaaaaactgtaaggaaataactgataaggaattggacaagaaaatgaaggagctcgccgccgtcatgagcgaccctgacctggaaactgagactatgtgcctccacgacgacgagtcgtgtcgctacgaagggcaagtcgctgtttaccaggatgtatacgcggttgacggaccgacaagtctctatcaccaagccaataagggagttagagtcgcctactggataggctttgacaccaccccttttatgtttaagaacttggctggagcatatccatcatactctaccaactgggccgacgaaaccgtgttaacggctcgtaacataggcctatgcagctctgacgttatggagcggtcacgtagagggatgtccattcttagaaagaagtatttgaaaccatccaacaatgttctattctctgttggctcgaccatctaccacgagaagagggacttactgaggagctggcacctgccgtctgtatttcacttacgtggcaagcaaaattacacatgtcggtgtgagactatagttagttgcgacgggtacgtcgttaaaagaatagctatcagtccaggcctgtatgggaagccttcaggctatgctgctacgatgcaccgcgagggattcttgtgctgcaaagtgacagacacattgaacggggagagggtctcttttcccgtgtgcacgtatgtgccagctacattgtgtgaccaaatgactggcatactggcaacagatgtcagtgcggacgacgcgcaaaaactgctggttgggctcaaccagcgtatagtcgtcaacggtcgcacccagagaaacaccaataccatgaaaaattaccttttgcccgtagtggcccaggcatttgctaggtgggcaaaggaatataaggaagatcaagaagatgaaaggccactaggactacgagatagacagttagtcatggggtgttgttgggcttttagaaggcacaagataacatctatttataagcgcccggatacccaaaccatcatcaaagtgaacagcgatttccactcattcgtgctgcccaggataggcagtaacacattggagatcgggctgagaacaagaatcaggaaaatgttagaggagcacaaggagccgtcacctctcattaccgccgaggacgtacaagaagctaagtgcgcagccgatgaggctaaggaggtgcgtgaagccgaggagttgcgcgcagctctaccacctttggcagctgatgttgaggagcccactctggaagccgatgtcgacttgatgttacaagaggctggggccggctcagtggagacacctcgtggcttgataaaggttaccagctacgatggcgaggacaagatcggctcttacgctgtgctttctccgcaggctgtactcaagagtgaaaaattatcttgcatccaccctctcgctgaacaagtcatagtgataacacactctggccgaaaagggcgttatgccgtggaaccataccatggtaaagtagtggtgccagagggacatgcaatacccgtccaggactttcaagctctgagtgaaagtgccaccattgtgtacaacgaacgtgagttcgtaaacaggtacctgcaccatattgccacacatggaggagcgctgaacactgatgaagaatattacaaaactgtcaagcccagcgagcacgacggcgaatacctgtacgacatcgacaggaaacagtgcgtcaagaaagaactagtcactgggctagggctcacaggcgagctggtggatcctcccttccatgaattcgcctacgagagtctgagaacacgaccagccgctccttaccaagtaccaaccataggggtgtatggcgtgccaggatcaggcaagtctggcatcattaaaagcgcagtcaccaaaaaagatctagtggtgagcgccaagaaagaaaactgtgcagaaattataagggacgtcaagaaaatgaaagggctggacgtcaatgccagaactgtggactcagtgctcttgaatggatgcaaacaccccgtagagaccctgtatattgacgaagcttttgcttgtcatgcaggtactctcagagcgctcatagccattataagacctaaaaaggcagtgctctgcggggatcccaaacagtgcggtttttttaacatgatgtgcctgaaagtgcattttaaccacgagatttgcacacaagtcttccacaaaagcatctctcgccgttgcactaaatctgtgacttcggtcgtctcaaccttgttttacgacaaaaaaatgagaacgacgaatccgaaagagactaagattgtgattgacactaccggcagtaccaaacctaagcaggacgatctcattctcacttgtttcagagggtgggtgaagcagttgcaaatagattacaaaggcaacgaaataatgacggcagctgcctctcaagggctgacccgtaaaggtgtgtatgccgttcggtacaaggtgaatgaaaatcctctgtacgcacccacctctgaacatgtgaacgtcctactgacccgcacggaggaccgcatcgtgtggaaaacactagccggcgacccatggataaaaacactgactgccaagtaccctgggaatttcactgccacgatagaggagtggcaagcagagcatgatgccatcatgaggcacatcttggagagaccggaccctaccgacgtcttccagaataaggcaaacgtgtgttgggccaaggctttagtgccggtgctgaagaccgctggcatagacatgaccactgaacaatggaacactgtggattattttgaaacggacaaagctcactcagcagagatagtattgaaccaactatgcgtgaggttctttggactcgatctggactccggtctattttctgcacccactgttccgttatccattaggaataatcactgggataactccccgtcgcctaacatgtacgggctgaataaagaagtggtccgtcagctctctcgcaggtacccacaactgcctcgggcagttgccactggaagagtctatgacatgaacactggtacactgcgcaattatgatccgcgcataaacctagtacctgtaaacagaagactgcctcatgctttagtcctccaccataatgaacacccacagagtgacttttcttcattcgtcagcaaattgaagggcagaactgtcctggtggtcggggaaaagttgtccgtcccaggcaaaatggttgactggttgtcagaccggcctgaggctaccttcagagctcggctggatttaggcatcccaggtgatgtgcccaaatatgacataatatttgttaatgtgaggaccccatataaataccatcactatcagcagtgtgaagaccatgccattaagcttagcatgttgaccaagaaagcttgtctgcatctgaatcccggcggaacctgtgtcagcataggttatggttacgctgacagggccagcgaaagcatcattggtgctatagcgcggcagttcaagttttcccgggtatgcaaaccgaaatcctcacttgaagagacggaagttctgtttgtattcattgggtacgatcgcaaggcccgtacgcacaatccttacaagctttcatcaaccttgaccaacatttatacaggttccagactccacgaagccggatgtgcaccctcatatcatgtggtgcgaggggatattgccacggccaccgaaggagtgattataaatgctgctaacagcaaaggacaacctggcggaggggtgtgcggagcgctgtataagaaattcccggaaagcttcgatttacagccgatcgaagtaggaaaagcgcgactggtcaaaggtgcagctaaacatatcattcatgccgtaggaccaaacttcaacaaagtttcggaggttgaaggtgacaaacagttggcagaggcttatgagtccatcgctaagattgtcaacgataacaattacaagtcagtagcgattccactgttgtccaccggcatcttttccgggaacaaagatcgactaacccaatcattgaaccatttgctgacagctttagacaccactgatgcagatgtagccatatactgcagggacaagaaatgggaaatgactctcaaggaagcagtggctaggagagaagcagtggaggagatatgcatatccgacgactcttcagtgacagaacctgatgcagagctggtgagggtgcatccgaagagttctttggctggaaggaagggctacagcacaagcgatggcaaaactttctcatatttggaagggaccaagtttcaccaggcggccaaggatatagcagaaattaatgccatgtggcccgttgcaacggaggccaatgagcaggtatgcatgtatatcctcggagaaagcatgagcagtattaggtcgaaatgccccgtcgaagagtcggaagcctccacaccacctagcacgctgccttgcttgtgcatccatgccatgactccagaaagagtacagcgcctaaaagcctcacgtccagaacaaattactgtgtgctcatcctttccattgccgaagtatagaatcactggtgtgcagaagatccaatgctcccagcctatattgttctcaccgaaagtgcctgcgtatattcatccaaggaagtatctcgtggaaacaccaccggtagacgagactccggagccatcggcagagaaccaatccacagaggggacacctgaacaaccaccacttataaccgaggatgagaccaggactagaacgcctgagccgatcatcatcgaagaggaagaagaggatagcataagtttgctgtcagatggcccgacccaccaggtgctgcaagtcgaggcagacattcacgggccgccctctgtatctagctcatcctggtccattcctcatgcatccgactttgatgtggacagtttatccatacttgacaccctggagggagctagcgtgaccagcggggcaacgtcagccgagactaactcttacttcgcaaagagtatggagtttctggcgcgaccggtgcctgcgcctcgaacagtattcaggaaccctccacatcccgctccgcgcacaagaacaccgtcacttgcacccagcagggcctgctcgagaaccagcctagtttccaccccgccaggcgtgaatagggtgatcactagagaggagctcgaggcgcttaccccgtcacgcactcctagcaggtcggtctcgagaaccagcctggtctccaacccgccaggcgtaaatagggtgattacaagagaggagtttgaggcgttcgtagcacaacaacaatgacggtttgatgcgggtgcatacatcttttcctccgacaccggtcaagggcatttacaacaaaaatcagtaaggcaaacggtgctatccgaagtggtgttggagaggaccgaattggagatttcgtatgccccgcgcctcgaccaagaaaaagaagaattactacgcaagaaattacagttaaatcccacacctgctaacagaagcagataccagtccaggaaggtggagaacatgaaagccataacagctagacgtattctgcaaggcctagggcattatttgaaggcagaaggaaaagtggagtgctaccgaaccctgcatcctgttcctttgtattcatctagtgtgaaccgtgccttttcaagccccaaggtcgcagtggaagcctgtaacgccatgttgaaagagaactttccgactgtggcttcttactgtattattccagagtacgatgcctatttggacatggttgacggagcttcatgctgcttagacactgccagtttttgccctgcaaagctgcgcagctttccaaagaaacactcctatttggaacccacaatacgatcggcagtgccttcagcgatccagaacacgctccagaacgtcctggcagctgccacaaaaagaaattgcaatgtcacgcaaatgagagaattgcccgtattggattcggcggcctttaatgtggaatgcttcaagaaatatgcgtgtaataatgaatattgggaaacgtttaaagaaaaccccatcaggcttactgaagaaaacgtggtaaattacattaccaaattaaaaggaccaaaagctgctgctctttttgcgaagacacataatttgaatatgttgcaggacataccaatggacaggtttgtaatggacttaaagagagacgtgaaagtgactccaggaacaaaacatactgaagaacggcccaaggtacaggtgatccaggctgccgatccgctagcaacagcgtatctgtgcggaatccaccgagagctggttaggagattaaatgcggtcctgcttccgaacattcatacactgtttgatatgtcggctgaagactttgacgctattatagccgagcacttccagcctggggattgtgttctggaaactgacatcgcgtcgtttgataaaagtgaggacgacgccatggctctgaccgcgttaatgattctggaagacttaggtgtggacgcagagctgttgacgctgattgaggcggctttcggcgaaatttcatcaatacatttgcccactaaaactaaatttaaattcggagccatgatgaaatctggaatgttcctcacactgtttgtgaacacagtcattaacattgtaatcgcaagcagagtgttgagagaacggctaaccggatcaccatgtgcagcattcattggagatgacaatatcgtgaaaggagtcaaatcggacaaattaatggcagacaggtgcgccacctggttgaatatggaagtcaagattatagatgctgtggtgggcgagaaagcgccttatttctgtggagggtttattttgtgtgactccgtgaccggcacagcgtgccgtgtggcagaccccctaaaaaggctgtttaagcttggcaaacctctggcagcagacgatgaacatgatgatgacaggagaagggcattgcatgaagagtcaacacgctggaaccgagtgggtattctttcagagctgtgcaaggcagtagaatcaaggtatgaaaccgtaggaacttccatcatagttatggccatgactactctagctagcagtgttaaatcattcagctacctgagaggggcccctataactctctacggctaacctgaatggactacgacatagtctagtccgccaagatatcgcaccatggaaaatatggaaaacgacgagaacatcgtggtgggccccaagcccttctaccccatcgaggaaggcagcgccggcacccagctgcggaagtacatggaaagatacgccaagctgggcgccattgccttcaccaacgccgtgaccggcgtggactacagctacgccgagtacctggaaaagagctgctgcctgggcaaggctctgcagaactacggcctggtggtggacggccggatcgccctgtgcagcgagaactgcgaggaattcttcatccccgtgatcgccggcctgttcatcggcgtgggcgtggctcccaccaacgagatctacaccctgcgggagctggtgcacagcctgggcatcagcaagcccaccatcgtgttcagcagcaagaagggcctggacaaagtcatcaccgtgcagaaaaccgtgaccaccatcaagaccatcgtgatcctggacagcaaggtggactaccggggctaccagtgcctggacaccttcatcaagcggaacaccccccctggcttccaggccagcagcttcaagaccgtggaggtggaccggaaagaacaggtggccctgatcatgaacagcagcggcagcaccggcctgcccaagggcgtgcagctgacccacgagaacaccgtgacccggttcagccacgccagggaccccatctacggcaaccaggtgtcccccggcaccgccgtgctgaccgtggtgcccttccaccacggcttcggcatgttcaccaccctgggctacctgatctgcggcttccgggtggtgatgctgaccaagttcgacgaggaaaccttcctgaaaaccctgcaggactacaagtgcacctacgtgattctggtgcccaccctgttcgccatcctgaacaagagcgagctgctgaacaagtacgacctgagcaacctggtggagatcgccagcggcggagcccccctgagcaaagaagtgggagaggccgtcgccaggcggttcaatctgcccggcgtgcggcagggctacggcctgaccgagacaaccagcgccatcatcatcacccccgagggcgacgacaagcctggagccagcggcaaggtggtgcccctgttcaaggccaaagtgatcgacctggacaccaagaagagcctgggccccaacagacggggcgaagtgtgcgtgaagggccccatgctgatgaagggctacgtgaacaaccccgaggccaccaaagagctgatcgacgaagagggctggctgcacaccggcgacatcggctactacgacgaagagaagcacttcttcatcgtggaccggctgaagagcctgatcaagtacaagggctatcaggtgccccctgccgagctggaaagcgtcctgctgcagcaccccagcatcttcgacgccggcgtggccggggtgccagatcctgtggccggcgagctgcctggcgccgtggtggtgctggaatccggcaagaacatgaccgagaaagaagtgatggactacgtcgccagccaggtgtccaacgccaagcggctgagaggcggcgtgagattcgtggacgaagtgccaaagggcctgaccggcaagatcgacggcagggccatccgggagatcctgaagaaacccgtggccaagatgtgattaattgatcgatacagcagcaattggcaagctgcttacatagaaggcgcgccgtttaaacggccggccttaattaagtaacgatacagcagcaattggcaagctgcttacatagaactcgcggcgattggcatgccgctttaaaatttttattttatttttcttttcttttccgaatcggattttgtttttaatatttcaaaaaaaaaaaaaaaaaaaaaaaaaaaaaaaaaaaaaaaa

SEQ ID NO: 29 - DNA, 10021 bp, Artificial Sequence
  Synthetic polynucleotide
  misc_feature: construct Alpha-R-DLP-2A-nsp-DLP-rFF
  misc_feature (1)...(18): T7 promoter
taatacgactcactatagataggcggcgcatgagagaagcccagaccaattacctacccaaataggagaaagttcacgttgacatcgaggaagacagcccattcctcagagctttgcagcggagcttcccgcagtttgaggtagaagccaagcaggtcactgataatgaccatgctaatgccagagcgttttcgcatctggcttcaaaactgatcgaaacggaggtggacccatccgacacgatccttgacattggaatagtcagcatagtacatttcatctgactaatactacaacaccaccaccatgaatagaggattctttaacatgctcggccgccgccccttcccggcccccactgccatgtggaggccgcggagaaggaggcaggcggccccgggaagcggagctactaacttcagcctgctgaagcaggctggagacgtggaggagaaccctggacctgagaaagttcacgttgacatcgaggaagacagcccattcctcagagctttgcagcggagcttcccgcagtttgaggtagaagccaagcaggtcactgataatgaccatgctaatgccagagcgttttcgcatctggcttcaaaactgatcgaaacggaggtggacccatccgacacgatccttgacattggaagtgcgcccgcccgcagaatgtattctaagcacaagtatcattgtatctgtccgatgagatgtgcggaagatccggacagattgtataagtatgcaactaagctgaagaaaaactgtaaggaaataactgataaggaattggacaagaaaatgaaggagctcgccgccgtcatgagcgaccctgacctggaaactgagactatgtgcctccacgacgacgagtcgtgtcgctacgaagggcaagtcgctgtttaccaggatgtatacgcggttgacggaccgacaagtctctatcaccaagccaataagggagttagagtcgcctactggataggctttgacaccaccccttttatgtttaagaacttggctggagcatatccatcatactctaccaactgggccgacgaaaccgtgttaacggctcgtaacataggcctatgcagctctgacgttatggagcggtcacgtagagggatgtccattcttagaaagaagtatttgaaaccatccaacaatgttctattctctgttggctcgaccatctaccacgagaagagggacttactgaggagctggcacctgccgtctgtatttcacttacgtggcaagcaaaattacacatgtcggtgtgagactatagttagttgcgacgggtacgtcgttaaaagaatagctatcagtccaggcctgtatgggaagccttcaggctatgctgctacgatgcaccgcgagggattcttgtgctgcaaagtgacagacacattgaacggggagagggtctcttttcccgtgtgcacgtatgtgccagctacattgtgtgaccaaatgactggcatactggcaacagatgtcagtgcggacgacgcgcaaaaactgctggttgggctcaaccagcgtatagtcgtcaacggtcgcacccagagaaacaccaataccatgaaaaattaccttttgcccgtagtggcccaggcatttgctaggtgggcaaaggaatataaggaagatcaagaagatgaaaggccactaggactacgagatagacagttagtcatggggtgttgttgggcttttagaaggcacaagataacatctatttataagcgcccggatacccaaaccatcatcaaagtgaacagcgatttccactcattcgtgctgcccaggataggcagtaacacattggagatcgggctgagaacaagaatcaggaaaatgttagaggagcacaaggagccgtcacctctcattaccgccgaggacgtacaagaagctaagtgcgcagccgatgaggctaaggaggtgcgtgaagccgaggagttgcgcgcagctctaccacctttggcagctgatgttgaggagcccactctggaagccgatgtcgacttgatgttacaagaggctggggccggctcagtggagacacctcgtggcttgataaaggttaccagctacgatggcgaggacaagatcggctcttacgctgtgctttctccgcaggctgtactcaagagtgaaaaattatcttgcatccaccctctcgctgaacaagtcatagtgataacacactctggccgaaaagggcgttatgccgtggaaccataccatggtaaagtagtggtgccagagggacatgcaatacccgtccaggactttcaagctctgagtgaaagtgccaccattgtgtacaacgaacgtgagttcgtaaacaggtacctgcaccatattgccacacatggaggagcgctgaacactgatgaagaatattacaaaactgtcaagcccagcgagcacgacggcgaatacctgtacgacatcgacaggaaacagtgcgtcaagaaagaactagtcactgggctagggctcacaggcgagctggtggatcctcccttccatgaattcgcctacgagagtctgagaacacgaccagccgctccttaccaagtaccaaccataggggtgtatggcgtgccaggatcaggcaagtctggcatcattaaaagcgcagtcaccaaaaaagatctagtggtgagcgccaagaaagaaaactgtgcagaaattataagggacgtcaagaaaatgaaagggctggacgtcaatgccagaactgtggactcagtgctcttgaatggatgcaaacaccccgtagagaccctgtatattgacgaagcttttgcttgtcatgcaggtactctcagagcgctcatagccattataagacctaaaaaggcagtgctctgcggggatcccaaacagtgcggtttttttaacatgatgtgcctgaaagtgcattttaaccacgagatttgcacacaagtcttccacaaaagcatctctcgccgttgcactaaatctgtgacttcggtcgtctcaaccttgttttacgacaaaaaaatgagaacgacgaatccgaaagagactaagattgtgattgacactaccggcagtaccaaacctaagcaggacgatctcattctcacttgtttcagagggtgggtgaagcagttgcaaatagattacaaaggcaacgaaataatgacggcagctgcctctcaagggctgacccgtaaaggtgtgtatgccgttcggtacaaggtgaatgaaaatcctctgtacgcacccacctctgaacatgtgaacgtcctactgacccgcacggaggaccgcatcgtgtggaaaacactagccggcgacccatggataaaaacactgactgccaagtaccctgggaatttcactgccacgatagaggagtggcaagcagagcatgatgccatcatgaggcacatcttggagagaccggaccctaccgacgtcttccagaataaggcaaacgtgtgttgggccaaggctttagtgccggtgctgaagaccgctggcatagacatgaccactgaacaatggaacactgtggattattttgaaacggacaaagctcactcagcagagatagtattgaaccaactatgcgtgaggttctttggactcgatctggactccggtctattttctgcacccactgttccgttatccattaggaataatcactgggataactccccgtcgcctaacatgtacgggctgaataaagaagtggtccgtcagctctctcgcaggtacccacaactgcctcgggcagttgccactggaagagtctatgacatgaacactggtacactgcgcaattatgatccgcgcataaacctagtacctgtaaacagaagactgcctcatgctttagtcctccaccataatgaacacccacagagtgacttttcttcattcgtcagcaaattgaagggcagaactgtcctggtggtcggggaaaagttgtccgtcccaggcaaaatggttgactggttgtcagaccggcctgaggctaccttcagagctcggctggatttaggcatcccaggtgatgtgcccaaatatgacataatatttgttaatgtgaggaccccatataaataccatcactatcagcagtgtgaagaccatgccattaagcttagcatgttgaccaagaaagcttgtctgcatctgaatcccggcggaacctgtgtcagcataggttatggttacgctgacagggccagcgaaagcatcattggtgctatagcgcggcagttcaagttttcccgggtatgcaaaccgaaatcctcacttgaagagacggaagttctgtttgtattcattgggtacgatcgcaaggcccgtacgcacaatccttacaagctttcatcaaccttgaccaacatttatacaggttccagactccacgaagccggatgtgcaccctcatatcatgtggtgcgaggggatattgccacggccaccgaaggagtgattataaatgctgctaacagcaaaggacaacctggcggaggggtgtgcggagcgctgtataagaaattcccggaaagcttcgatttacagccgatcgaagtaggaaaagcgcgactggtcaaaggtgcagctaaacatatcattcatgccgtaggaccaaacttcaacaaagtttcggaggttgaaggtgacaaacagttggcagaggcttatgagtccatcgctaagattgtcaacgataacaattacaagtcagtagcgattccactgttgtccaccggcatcttttccgggaacaaagatcgactaacccaatcattgaaccatttgctgacagctttagacaccactgatgcagatgtagccatatactgcagggacaagaaatgggaaatgactctcaaggaagcagtggctaggagagaagcagtggaggagatatgcatatccgacgactcttcagtgacagaacctgatgcagagctggtgagggtgcatccgaagagttctttggctggaaggaagggctacagcacaagcgatggcaaaactttctcatatttggaagggaccaagtttcaccaggcggccaaggatatagcagaaattaatgccatgtggcccgttgcaacggaggccaatgagcaggtatgcatgtatatcctcggagaaagcatgagcagtattaggtcgaaatgccccgtcgaagagtcggaagcctccacaccacctagcacgctgccttgcttgtgcatccatgccatgactccagaaagagtacagcgcctaaaagcctcacgtccagaacaaattactgtgtgctcatcctttccattgccgaagtatagaatcactggtgtgcagaagatccaatgctcccagcctatattgttctcaccgaaagtgcctgcgtatattcatccaaggaagtatctcgtggaaacaccaccggtagacgagactccggagccatcggcagagaaccaatccacagaggggacacctgaacaaccaccacttataaccgaggatgagaccaggactagaacgcctgagccgatcatcatcgaagaggaagaagaggatagcataagtttgctgtcagatggcccgacccaccaggtgctgcaagtcgaggcagacattcacgggccgccctctgtatctagctcatcctggtccattcctcatgcatccgactttgatgtggacagtttatccatacttgacaccctggagggagctagcgtgaccagcggggcaacgtcagccgagactaactcttacttcgcaaagagtatggagtttctggcgcgaccggtgcctgcgcctcgaacagtattcaggaaccctccacatcccgctccgcgcacaagaacaccgtcacttgcacccagcagggcctgctcgagaaccagcctagtttccaccccgccaggcgtgaatagggtgatcactagagaggagctcgaggcgcttaccccgtcacgcactcctagcaggtcggtctcgagaaccagcctggtctccaacccgccaggcgtaaatagggtgattacaagagaggagtttgaggcgttcgtagcacaacaacaatgacggtttgatgcgggtgcatacatcttttcctccgacaccggtcaagggcatttacaacaaaaatcagtaaggcaaacggtgctatccgaagtggtgttggagaggaccgaattggagatttcgtatgccccgcgcctcgaccaagaaaaagaagaattactacgcaagaaattacagttaaatcccacacctgctaacagaagcagataccagtccaggaaggtggagaacatgaaagccataacagctagacgtattctgcaaggcctagggcattatttgaaggcagaaggaaaagtggagtgctaccgaaccctgcatcctgttcctttgtattcatctagtgtgaaccgtgccttttcaagccccaaggtcgcagtggaagcctgtaacgccatgttgaaagagaactttccgactgtggcttcttactgtattattccagagtacgatgcctatttggacatggttgacggagcttcatgctgcttagacactgccagtttttgccctgcaaagctgcgcagctttccaaagaaacactcctatttggaacccacaatacgatcggcagtgccttcagcgatccagaacacgctccagaacgtcctggcagctgccacaaaaagaaattgcaatgtcacgcaaatgagagaattgcccgtattggattcggcggcctttaatgtggaatgcttcaagaaatatgcgtgtaataatgaatattgggaaacgtttaaagaaaaccccatcaggcttactgaagaaaacgtggtaaattacattaccaaattaaaaggaccaaaagctgctgctctttttgcgaagacacataatttgaatatgttgcaggacataccaatggacaggtttgtaatggacttaaagagagacgtgaaagtgactccaggaacaaaacatactgaagaacggcccaaggtacaggtgatccaggctgccgatccgctagcaacagcgtatctgtgcggaatccaccgagagctggttaggagattaaatgcggtcctgcttccgaacattcatacactgtttgatatgtcggctgaagactttgacgctattatagccgagcacttccagcctggggattgtgttctggaaactgacatcgcgtcgtttgataaaagtgaggacgacgccatggctctgaccgcgttaatgattctggaagacttaggtgtggacgcagagctgttgacgctgattgaggcggctttcggcgaaatttcatcaatacatttgcccactaaaactaaatttaaattcggagccatgatgaaatctggaatgttcctcacactgtttgtgaacacagtcattaacattgtaatcgcaagcagagtgttgagagaacggctaaccggatcaccatgtgcagcattcattggagatgacaatatcgtgaaaggagtcaaatcggacaaattaatggcagacaggtgcgccacctggttgaatatggaagtcaagattatagatgctgtggtgggcgagaaagcgccttatttctgtggagggtttattttgtgtgactccgtgaccggcacagcgtgccgtgtggcagaccccctaaaaaggctgtttaagcttggcaaacctctggcagcagacgatgaacatgatgatgacaggagaagggcattgcatgaagagtcaacacgctggaaccgagtgggtattctttcagagctgtgcaaggcagtagaatcaaggtatgaaaccgtaggaacttccatcatagttatggccatgactactctagctagcagtgttaaatcattcagctacctgagaggggcccctataactctctacggctaacctgaatggactacgacatagtctagtccgccaagatatcgcaccatagtcagcatagtacatttcatctgactaatactacaacaccaccaccatgaatagaggattctttaacatgctcggccgccgccccttcccggcccccactgccatgtggaggccgcggagaaggaggcaggcggccccgatgatggaaaatatggaaaacgacgagaacatcgtggtgggccccaagcccttctaccccatcgaggaaggcagcgccggcacccagctgcggaagtacatggaaagatacgccaagctgggcgccattgccttcaccaacgccgtgaccggcgtggactacagctacgccgagtacctggaaaagagctgctgcctgggcaaggctctgcagaactacggcctggtggtggacggccggatcgccctgtgcagcgagaactgcgaggaattcttcatccccgtgatcgccggcctgttcatcggcgtgggcgtggctcccaccaacgagatctacaccctgcgggagctggtgcacagcctgggcatcagcaagcccaccatcgtgttcagcagcaagaagggcctggacaaagtcatcaccgtgcagaaaaccgtgaccaccatcaagaccatcgtgatcctggacagcaaggtggactaccggggctaccagtgcctggacaccttcatcaagcggaacaccccccctggcttccaggccagcagcttcaagaccgtggaggtggaccggaaagaacaggtggccctgatcatgaacagcagcggcagcaccggcctgcccaagggcgtgcagctgacccacgagaacaccgtgacccggttcagccacgccagggaccccatctacggcaaccaggtgtcccccggcaccgccgtgctgaccgtggtgcccttccaccacggcttcggcatgttcaccaccctgggctacctgatctgcggcttccgggtggtgatgctgaccaagttcgacgaggaaaccttcctgaaaaccctgcaggactacaagtgcacctacgtgattctggtgcccaccctgttcgccatcctgaacaagagcgagctgctgaacaagtacgacctgagcaacctggtggagatcgccagcggcggagcccccctgagcaaagaagtgggagaggccgtcgccaggcggttcaatctgcccggcgtgcggcagggctacggcctgaccgagacaaccagcgccatcatcatcacccccgagggcgacgacaagcctggagccagcggcaaggtggtgcccctgttcaaggccaaagtgatcgacctggacaccaagaagagcctgggccccaacagacggggcgaagtgtgcgtgaagggccccatgctgatgaagggctacgtgaacaaccccgaggccaccaaagagctgatcgacgaagagggctggctgcacaccggcgacatcggctactacgacgaagagaagcacttcttcatcgtggaccggctgaagagcctgatcaagtacaagggctatcaggtgccccctgccgagctggaaagcgtcctgctgcagcaccccagcatcttcgacgccggcgtggccggggtgccagatcctgtggccggcgagctgcctggcgccgtggtggtgctggaatccggcaagaacatgaccgagaaagaagtgatggactacgtcgccagccaggtgtccaacgccaagcggctgagaggcggcgtgagattcgtggacgaagtgccaaagggcctgaccggcaagatcgacggcagggccatccgggagatcctgaagaaacccgtggccaagatgtgattaattgatcgatacagcagcaattggcaagctgcttacatagaaggcgcgccgtttaaacggccggccttaattaagtaacgatacagcagcaattggcaagctgcttacatagaactcgcggcgattggcatgccgctttaaaatttttattttatttttcttttcttttccgaatcggattttgtttttaatatttcaaaaaaaaaaaaaaaaaaaaaaaaaaaaaaaaaaaaaaaa

SEQ ID NO: 30 - DNA, 1150 bp, Artificial Sequence
  Synthetic polynucleotide
  misc_feature: g-block for Alpha-R-DLP-2A-rFF
tctacggctaacctgaatggactacgacatagtctagtccgccaagatatcgcaccatagtcagcatagtacatttcatctgactaatactacaacaccaccaccatgaatagaggattctttaacatgctcggccgccgccccttcccggcccccactgccatgtggaggccgcggagaaggaggcaggcggccccgggaagcggagctactaacttcagcctgctgaagcaggctggagacgtggaggagaaccctggacctatggaaaatatggaaaacgacgagaacatcgtggtgggccccaagcccttctaccccatcgaggaaggcagcgccggcacccagctgcggaagtacatggaaagatacgccaagctgggcgccattgccttcaccaacgccgtgaccggcgtggactacagctacgccgagtacctggaaaagagctgctgcctgggcaaggctctgcagaactacggcctggtggtggacggccggatcgccctgtgcagcgagaactgcgaggaattcttcatccccgtgatcgccggcctgttcatcggcgtgggcgtggctcccaccaacgagatctacaccctgcgggagctggtgcacagcctgggcatcagcaagcccaccatcgtgttcagcagcaagaagggcctggacaaagtcatcaccgtgcagaaaaccgtgaccaccatcaagaccatcgtgatcctggacagcaaggtggactaccggggctaccagtgcctggacaccttcatcaagcggaacaccccccctggcttccaggccagcagcttcaagaccgtggaggtggaccggaaagaacaggtggccctgatcatgaacagcagcggcagcaccggcctgcccaagggcgtgcagctgacccacgagaacaccgtgacccggttcagccacgccagggaccccatctacggcaaccaggtgtcccccggcaccgccgtgctgaccgtggtgcccttccaccacggcttcggcatgttcaccaccctgggctacctgatctgcggcttccgggtggtgatgctgaccaagttcgacgaggaaaccttcctgaaaaccctgcaggactacaagtgcacctacgtgattctggtgcccaccctgttcgcca

SEQ ID NO: 31 - DNA, 1150 bp, Artificial Sequence; identical to SEQ ID NO: 30
  Synthetic polynucleotide
  misc_feature: g-block for Alpha-R-DLP-2A-nsp-DLP-2A-rFF

SEQ ID NO: 32 - DNA, 25 bp, Artificial Sequence
  Synthetic polynucleotide
  misc_feature: primer Alpha-3'nsp4-F
  misc_feature: RP123
ggctgtttaagcttggcaaacctct

SEQ ID NO: 33 - DNA, 23 bp, Artificial Sequence
  Synthetic polynucleotide
  misc_feature: primer Alpha-3'nsp4-F
  misc_feature: rFF-seq1
agcgagaactgcgaggaattctt

SEQ ID NO: 34 - DNA, 12342 bp, Artificial Sequence
  Synthetic polypeptide
  misc_feature: Construct rEx-rFF
gctcgaagtgtgtatggtgccatatacggctcaccaccatatacactgcaagaattactattcttgtgggcccctctcggtaaatcctagagggctttcctctcgttattgcgagattcgtcgttagataacggcaagttccctttcttactatcctattttcatcttgtggcttgacgggtcactgccatcgtcgtcgatctctatcaactacccttgcgactatggcaaccttctccgctactggatttggagggagttttgttagggactggtccctggacttacccgacgcttgtgagcatggcgcgggattgtgctgcgaagtggacggctccaccttatgcgccgagtgttttcgcggttgcgaaggaatggagcaatgtcctggcttgttcatgggactgttaaaactggcttcgccagttccagtgggacataagttcctgattggttggtatcgagctgccaaagtcaccgggcgttacaatttccttgagctgttgcaacaccctgctttcgcccagctgcgtgtggttgatgctaggttagccattgaagaggcaagtgtgtttatttccactgaccacgcgtctgctaagcgtttccctggcgctagatttgcgctgacaccggtgtatgctaacgcttgggttgtgagcccggctgctaacagtttgatagtgaccactgaccaggaacaagatgggttctgctggttaaaacttttgccacctgaccgccgtgaggctggtttgcggttgtattacaaccattaccgcgaacaaaggaccgggtggctgtctaaaacaggacttcgcttatggcttggagacctgggtttgggcatcaatgcgagctctggagggctgaaattccacattatgaggggttcgcctcagcgagcttggcatatcacaacacgcagctgcaagctgaagagctactacgtttgtgacatctctgaagcagactggtcctgtttgcctgctggcaactacggcggctacaatccaccaggggacggagcttgcggttacaggtgcttggccttcatgaatggcgccactgttgtgtcggctggttgcagttctgacttgtggtgtgatgatgagttggcttatcgagtctttcaattgtcacccacgttcacggttaccatcccaggtgggcgagtttgtccgaatgccaagtacgcaatgatttgtgacaagcagcactggcgcgtcaaacgtgcaaagggcgtcggcctgtgtctcgatgaaagctgtttcaggggcatctgcaattgccaacgcatgagtggaccaccacctgcacccgtgtcagccgccgtgttagatcacatactggaggcggcgacgtttggcaacgttcgcgtggttacacctgaagggcagccacgccccgtaccagcgccgcgagttcgtcccagcgccaactcttctggagatgtcaaagatccggcgcccgttccgccagtaccaaaaccaaggaccaagcttgccacaccgaacccaactcaggcgcccatcccagcaccgcgcacgcgacttcaaggggcctcaacacaggagccactggcgagtgcaggagttgcttctgactcggcacctaaatggcgtgtggccaaaactgtgtacagctccgcggagcgctttcggaccgaactggtacaacgtgctcggtccgttggggacgttcttgttcaagcgctaccgctcaaaaccccagcagtgcagcggtataccatgactctgaagatgatgcgttcacgcttcagttggcactgcgacgtgtggtaccctttggctgtaatcgcttgtttgctccctatatggccatctcttgctttgctccttagctttgccattgggttgatacccagtgtgggcaataatgttgttctgacagcgcttctggtttcatcagctaattatgttgcgtcaatggaccatcaatgtgaaggtgcggcttgcttagccttgctggaagaagaacactattatagagcggtccgttggcgcccgattacaggcgcgctgtcgcttgtgctcaatttactggggcaggtaggctatgtagctcgttccacctttgatgcagcttatgttccttgcactgtgttcgatctttgcagctttgctattctgtacctctgccgcaatcgttgctggagatgcttcggacgctgtgtgcgagttgggcctgccacgcatgttttgggctccaccgggcaacgagtttccaaactggcgctcattgatttgtgtgaccacttttcaaagcccaccatcgatgttgtgggcatggcaactggttggagcggatgttacacaggaaccgccgcaatggagcgtcagtgtgcctctacggtggaccctcactcgttcgaccagaagaaggcaggagcgactgtttacctcaccccccctgtcaacagcgggtcagcgctgcagtgcctcaatgtcatgtggaagcgaccaattgggtccactgtccttggggaacaaacaggagctgttgtgacggcggtcaagagtatctctttctcacctccctgctgcgtctctaccactttgcccacccgacccggtgtgaccgttgtcgaccatgctctttacaaccggttgactgcttcaggggtcgatcccgctttattgcgtgttgggcaaggtgattttctaaaacttaatccggggttccggctgataggtggatggatttatgggatatgctattttgtgttggtggttgtgtcaacttttacctgcttacctatcaaatgtggcattggcacccgcgaccctttctgccgcagagtgttttctgtacccgtcaccaagacccaagagcactgccatgctggaatgtgtgctagcgctgaaggcatctctctggactctctggggttaactcagttacaaagttactggatcgcagccgtcactagcggattagtgatcttgttggtctgccaccgcctggccatcagcgccttggacttgttgactctagcttcccctttagtgttgcttgtgttcccttgggcatctgtggggcttttacttgcttgcagtctcgctggtgctgctgtgaaaatacagttgttggcgacgctttttgtgaatctattctttccccaagctacccttgtcactatgggatactgggcgtgcgtggcggctttggccgtttacagtttgatgggcttgcgagtgaaagtgaatgtgcccatgtgtgtgacacctgcccattttctgctgctggcgaggtcagctggacagtcaagagagcagatgctccgggtcagcgctgctgcccccaccaattcactgcttggagtggctcgtgattgttatgtcacaggcacaactcggctgtacatacccaaggaaggcgggatggtgtttgaagggctattcaggtcaccgaaggcgcgcggcaacgtcggcttcgtggctggtagcagctacggcacagggtcagtgtggaccaggaacaacgaggtcgtcgtactgacagcgtcacacgtggttggccgcgctaacatggccactctgaagatcggtgacgcaatgctgactctgactttcaaaaagaatggcgacttcgccgaggcagtgacgacacagtccgagctcccaggcaattggccacagttgcatttcgcccaaccaacaaccgggcccgcttcatggtgcactgccacaggagatgaagaaggcttgctcagtggcgaggtttgtctggcgtggactactagtggcgactctggatctgcagtggttcagggtgacgctgtggtaggggtccacaccggttcgaacacaagtggtgttgcctacgtgaccaccccaagcggaaaactccttggcgccgacaccgtgactttgtcatcactgtcaaagcatttcacaggccctttgacatcaatcccgaaggacatccctgacaacattattgccgatgttgatgctgttcctcgttctctggccatgctgattgatggcttatccaatagagagagcagcctttctggacctcagttgttgttaattgcttgttttatgtggtcttatcttaaccaacctgcttacttgccttatgtgctgggcttctttgccgctaacttcttcctgccaaaaagtgttggccgccctgtggtcactgggcttctatggttgtgctgcctcttcacaccgctttccatgcgcttgtgcttgttccatctggtctgtgctaccgtcacgggaaacgtgatatctttgtggttctacatcactgccgctggcacgtcttacctttctgagatgtggttcggaggctatcccaccatgttgtttgtgccacggttcctagtgtaccagttccccggctgggctattggcacagtactagcggtatgcagcatcaccatgctggctgctgccctcggtcacaccctgttactggatgtgttctccgcctcaggtcgctttgacaggactttcatgatgaaatacttcctggagggaggagtgaaagagagtgtcaccgcctcagtcacccgcgcttatggcaaaccaattacccaggagagtctcactgcaacattagctgccctcactgatgatgacttccaattcctctctgatgtgcttgactgtcgggccgtccgatcggcaatgaatctgcgtgccgctctcacaagttttcaagtggcgcagtatcgtaacatccttaatgcatccttgcaagtcgatcgtgacgctgctcgtagtcgcagactaatggcaaaactggctgattttgcggttgaacaagaagtaacagctggagaccgtgttgtggttatcgacggtctggaccgcatggctcacttcaaagacgatttggtgctggttcctttgaccaccaaagtagtaggcggttctaggtgcaccatttgtgacgtcgttaaggaagaagccaatgacaccccagttaagccaatgcccagcaggagacgccgcaagggcctgcctaaaggtgctcagttggagtgggaccgtcaccaggaagagaagaggaacgccggtgatgatgattttgcggtctcgaatgattatgtcaagagagtgccaaagtactgggatcccagcgacacccgaggcacgacagtgaaaatcgccggcactacctatcagaaagtggttgactattcaggcaatgtgcattacgtggagcatcaggaagatctgctagactacgtgctgggcaaggggagctatgaaggcctagatcaggacaaagtgttggacctcacaaacatgcttaaagtggaccccacggagctctcctccaaagacaaagccaaggcgcgtcagcttgctcatctgctgttggatctggctaacccagttgaggcagtgaatcagttaaactgagagcgccccacatctttcccggcgatgtggggcgtcggacctttgctgactctaaagacaagggtttcgtggctctacacagtcgcacaatgtttttagctgcccgggactttttatttaacatcaaatttgtgtgcgacgaagagttcacaaagaccccaaaagacacactgcttgggtacgtacgcgcctgccctggttactggtttattttccgtcgtacgcaccggtcgctgattgatgcatactgggacagtatggagtgcgtttacgcgcttcccaccatatctgattttgatgtgagcccaggtgacgtcgcagtgacgggcgagcgatgggattttgaatctcccggaggaggccgtgcaaaacgtctcacagctgatctggtgcacgcttttcaagggttccacggagcctcttattcctatgatgacaaggtggcagctgctgtcagtggtgacccgtatcggtcggacggcgtcttgtataacacccgttggggcaacattccatattctgtcccaaccaatgctttggaagccacagcttgctaccgtgctggatgtgaggccgttaccgacgggaccaacgtcatcgcaacaattgggcccttcccggagcaacaacccataccggacatcccaaagagcgtgcttgacaactgcgctgacatcagctgtgacgctttcatagcgcccgctgcagagacagccctgtgtggagatttagagaaatacaacctatccacgcagggttttgtgttgcctagtgttttctccatggtgcgggcgtacttaaaagaggagattggagacgctccaccactctacttgccatctactgtaccatctaaaaattcacaagccggaattaacggcgctgagtttcctacaaagtctttacagagctactgtttgattgatgacatggtgtcacagtccatgaaaagcaatctacaaaccgccaccatggcgacttgtaaacggcaatactgttccaaatacaagattaggagcattctgggcaccaacaattacattggcctaggtttgcgtgcctgcctttcgggggttacggccgcattccaaaaagctggaaaggatgggtcaccgatttatttgggcaagtcaaaattcgacccgataccagctcctgacaagtactgccttgaaacagacctggagagttgtgatcgctccaccccggctttggtgcgttggttcgctactaatcttatttttgagctagctggccagcccgagttggtgcacagctacgtgttgaattgctgtcacgatctagttgtggcgggtagtgtagcattcaccaaacgcgggggtttgtcatctggagaccctatcacttccatttccaataccatctattcattggtgctgtacacccagcacatgttgctatgtggacttgaaggctatttcccagagattgcagaaaaatatcttgatggcagcctggagctgcgggacatgttcaagtacgttcgagtgtacatctactcggacgatgtggttctaaccacacccaaccagcattacgcggccagctttgaccgctgggtcccccacctgcaggcgctgctaggtttcaaggttgacccaaagaaaactgtgaacaccagctccccttcctttttgggctgccggttcaagcaagtggacggcaagtgttatctagccagtcttcaggaccgcgttacacgctctctgttataccacattggtgcaaagaatccctcagagtactatgaagctgctgtttccatctttaaggactccattatctgctgtgatgaagactggtggacggacctccatcgacgtatcagtggcgctgcgcgtaccgacggagttgagttccccaccattgaaatgttaacatccttccgcaccaagcagtatgagagtgccgtgtgcacagtttgtggggccgcccccgtggccaagtctgcttgtggagggtggttctgtggcaattgtgtcccgtaccacgcgggtcattgtcacacaacctcgctcttcgccaactgcgggcacgacatcatgtaccgctccacttactgcacaatgtgtgagggttccccaaaacagatggtaccaaaagtgcctcacccgatcctggatcatttgctgtgccacattgattacggcagtaaagaggaactaactctggtagtggcggatggtcgaacaacatcaccgcccgggcgctacaaagtgggtcacaaggtagtcgccgtggttgcagatgtgggaggcaacattgtgtttgggtgcggtcctggatcacacatcgcagtaccacttcaggatacgctcaagggcgtggtggtgaataaagctctgaagaacgccgccgcctctgagtacgtggaaggaccccctgggagtgggaagacttttcacctggtcaaagatgtgctagccgtggtcggtagcgcgaccttggttgtgcccacccacgcgtccatgctggactgcatcaacaagctcaaacaagcgggcgccgatccatactttgtggtgcccaagtatacagttcttgactttccccggcctggcagtggaaacatcacagtgcgactgccacaggtcggaaccagtgagggagaaacctttgtggatgaggtggcctacttctcaccagtggatctggcgcgcattttaacccagggtcgagtcaagggttacggtgatttaaatcagctcgggtgcgtcggacccgcgagcgtgccacgtaacctttggctccgacattttgtcagcctggagcccttgcgagtgtgccatcgattcggcgctgctgtgtgtgatttgatcaagggcatttatccttattatgagccagctccacataccactaaagtggtgtttgtgccaaatccagactttgagaaaggtgtagtcatcaccgcctaccacaaagatcgcggtcttggtcaccgcacaattgattcaattcaaggctgtacattccctgttgtgactcttcgactgcccacaccccaatcactgacgcgcccgcgcgcagttgtggcggttactagggcgtctcaggaattatacatctacgacccctttgatcagcttagcgggttgttgaagttcaccaaggaagcagaggcgcaggacttgatccatggcccacctacagcatgccacctgggccaagaaattgacctttggtccaatgagggcctcgaatattacaaggaagtcaacctgctgtacacacacgtccccatcaaggatggtgtaatacacagttaccctaattgtggccctgcctgtggctgggaaaagcaatccaacaaaatttcgtgcctcccgagagtggcacaaaatttgggctaccactattccccagacttaccaggattttgccccataccaaaagaactcgctgagcattggcccgtagtgtccaatgatagatacccgaattgcttgcaaattaccttacagcaagtatgtgaactcagtaaaccgtgctcagcgggctatatggttggacaatcggttttcgtgcagacgcctggtgtgacatcttactggcttactgaatgggtcgacggcaaagcgcgtgctctaccagattccttattctcgtccggtaggttcgagactaacagccgcgctttcctcgatgaagccgaggaaaagtttgccgccgctcaccctcatgcctgtttgggagaaattaataagtccaccgtgggaggatcccacttcatcttttcccaatatttaccaccattgctacccgcagacgctgttgccctggtaggtgcttcattggctgggaaagctgctaaagctgcttgcagcgttgttgatgtctatgctccatcatttgaaccttatctacaccctgagacactgagtcgcgtgtacaagattatgatcgatttcaagccgtgtaggcttatggtgtggagaaacgcgaccttttatgtccaagagggtgttgatgcagttacatcagcactagcagctgtgtccaaactcatcaaagtgccggccaatgagcctgtttcattccatgtggcatcagggtacagaaccaacgcgctggtagcgccccaggctaaaatttcaattggagcctacgccgccgagtgggcactgtcaactgaaccgccacctgctggttatgcgatcgtgcggcgatatattgtaaagaggctcctcagctcaacagaagtgttcttgtgccgcaggggtgttgtgtcttccacctcagtgcagaccatttgtgcactagagggatgtaaacctctgttcaacttcttacaaattggttcagtcattgggcccgtgtgactctagagtggacctgttcccatcccccgctcaactactcaggtagtggttcgcggcaacgggtacaccgcagttggtaacaagcttgtcgatggaaaatatggaaaacgacgagaacatcgtggtgggccccaagcccttctaccccatcgaggaaggcagcgccggcacccagctgcggaagtacatggaaagatacgccaagctgggcgccattgccttcaccaacgccgtgaccggcgtggactacagctacgccgagtacctggaaaagagctgctgcctgggcaaggctctgcagaactacggcctggtggtggacggccggatcgccctgtgcagcgagaactgcgaggaattcttcatccccgtgatcgccggcctgttcatcggcgtgggcgtggctcccaccaacgagatctacaccctgcgggagctggtgcacagcctgggcatcagcaagcccaccatcgtgttcagcagcaagaagggcctggacaaagtcatcaccgtgcagaaaaccgtgaccaccatcaagaccatcgtgatcctggacagcaaggtggactaccggggctaccagtgcctggacaccttcatcaagcggaacaccccccctggcttccaggccagcagcttcaagaccgtggaggtggaccggaaagaacaggtggccctgatcatgaacagcagcggcagcaccggcctgcccaagggcgtgcagctgacccacgagaacaccgtgacccggttcagccacgccagggaccccatctacggcaaccaggtgtcccccggcaccgccgtgctgaccgtggtgcccttccaccacggcttcggcatgttcaccaccctgggctacctgatctgcggcttccgggtggtgatgctgaccaagttcgacgaggaaaccttcctgaaaaccctgcaggactacaagtgcacctacgtgattctggtgcccaccctgttcgccatcctgaacaagagcgagctgctgaacaagtacgacctgagcaacctggtggagatcgccagcggcggagcccccctgagcaaagaagtgggagaggccgtcgccaggcggttcaatctgcccggcgtgcggcagggctacggcctgaccgagacaaccagcgccatcatcatcacccccgagggcgacgacaagcctggagccagcggcaaggtggtgcccctgttcaaggccaaagtgatcgacctggacaccaagaagagcctgggccccaacagacggggcgaagtgtgcgtgaagggccccatgctgatgaagggctacgtgaacaaccccgaggccaccaaagagctgatcgacgaagagggctggctgcacaccggcgacatcggctactacgacgaagagaagcacttcttcatcgtggaccggctgaagagcctgatcaagtacaagggctatcaggtgccccctgccgagctggaaagcgtcctgctgcagcaccccagcatcttcgacgccggcgtggccggggtgccagatcctgtggccggcgagctgcctggcgccgtggtggtgctggaatccggcaagaacatgaccgagaaagaagtgatggactacgtcgccagccaggtgtccaacgccaagcggctgagaggcggcgtgagattcgtggacgaagtgccaaagggcctgaccggcaagatcgacggcagggccatccgggagatcctgaagaaacccgtggccaagatgtgattataactcgagggagccatagattcattttgtggtgacgggattttaggtgagtatctagattactttattctgtccgtcccactcttgctgttgcttactaggtatgtagcatctgggttagtgtatgttttgactgccttgttctattcctttgtattagcagcttatatttggtttgttatagttggaagagccttttctactgcttatgcttttgtgcttttggctgcttttctgttattagtaatgaggatgattgtgggtatgatgcctcgtcttcggtccattttcaaccatcgccaactggtggtagctgattttgtggacacacctagtggacctgttcccatcccccgcccaaccactcaggtagtggttcgcggcaacgggtacaccgcagttggtaacaagcttgtcgatggcgtcaagacgatcacgtccgcaggccgcctcttttcgaaacggacggcggcgacagcctacaagctacaatgacctactgcgcatgtttggtcagatgcgggtccgcaaaccgcccgcgcaacccactcaggctattattgcagagcctggagaccttaggcatgatttaaatcaacaggagcgcgccaccctttcgtcgaacgtacaacggttcttcatgattgggcatggttcactcactgcagatgccggaggactcacgtacaccgtcagttgggttcctaccaaacaaatccagcgcaaagttgcgcctccagcagggccgtaagacgtggatattctcctgtgtggcgtcatgttgaagtagttattagccacccaggaaccaaaaaaaaaaaaaaaaaaaaaaaaaaaaaaaaaaaaaaaa

SEQ ID NO: 35 - DNA, 8554 bp, Artificial Sequence
  Synthetic polypeptide
  misc_feature: Construct Alpha-R-eGFP
ataggcggcgcatgagagaagcccagaccaattacctacccaaaatggagaaagttcacgttgacatcgaggaagacagcccattcctcagagctttgcagcggagcttcccgcagtttgaggtagaagccaagcaggtcactgataatgaccatgctaatgccagagcgttttcgcatctggcttcaaaactgatcgaaacggaggtggacccatccgacacgatccttgacattggaagtgcgcccgcccgcagaatgtattctaagcacaagtatcattgtatctgtccgatgagatgtgcggaagatccggacagattgtataagtatgcaactaagctgaagaaaaactgtaaggaaataactgataaggaattggacaagaaaatgaaggagctcgccgccgtcatgagcgaccctgacctggaaactgagactatgtgcctccacgacgacgagtcgtgtcgctacgaagggcaagtcgctgtttaccaggatgtatacgcggttgacggaccgacaagtctctatcaccaagccaataagggagttagagtcgcctactggataggctttgacaccaccccttttatgtttaagaacttggctggagcatatccatcatactctaccaactgggccgacgaaaccgtgttaacggctcgtaacataggcctatgcagctctgacgttatggagcggtcacgtagagggatgtccattcttagaaagaagtatttgaaaccatccaacaatgttctattctctgttggctcgaccatctaccacgagaagagggacttactgaggagctggcacctgccgtctgtatttcacttacgtggcaagcaaaattacacatgtcggtgtgagactatagttagttgcgacgggtacgtcgttaaaagaatagctatcagtccaggcctgtatgggaagccttcaggctatgctgctacgatgcaccgcgagggattcttgtgctgcaaagtgacagacacattgaacggggagagggtctcttttcccgtgtgcacgtatgtgccagctacattgtgtgaccaaatgactggcatactggcaacagatgtcagtgcggacgacgcgcaaaaactgctggttgggctcaaccagcgtatagtcgtcaacggtcgcacccagagaaacaccaataccatgaaaaattaccttttgcccgtagtggcccaggcatttgctaggtgggcaaaggaatataaggaagatcaagaagatgaaaggccactaggactacgagatagacagttagtcatggggtgttgttgggcttttagaaggcacaagataacatctatttataagcgcccggatacccaaaccatcatcaaagtgaacagcgatttccactcattcgtgctgcccaggataggcagtaacacattggagatcgggctgagaacaagaatcaggaaaatgttagaggagcacaaggagccgtcacctctcattaccgccgaggacgtacaagaagctaagtgcgcagccgatgaggctaaggaggtgcgtgaagccgaggagttgcgcgcagctctaccacctttggcagctgatgttgaggagcccactctggaagccgatgtcgacttgatgttacaagaggctggggccggctcagtggagacacctcgtggcttgataaaggttaccagctacgatggcgaggacaagatcggctcttacgctgtgctttctccgcaggctgtactcaagagtgaaaaattatcttgcatccaccctctcgctgaacaagtcatagtgataacacactctggccgaaaagggcgttatgccgtggaaccataccatggtaaagtagtggtgccagagggacatgcaatacccgtccaggactttcaagctctgagtgaaagtgccaccattgtgtacaacgaacgtgagttcgtaaacaggtacctgcaccatattgccacacatggaggagcgctgaacactgatgaagaatattacaaaactgtcaagcccagcgagcacgacggcgaatacctgtacgacatcgacaggaaacagtgcgtcaagaaagaactagtcactgggctagggctcacaggcgagctggtggatcctcccttccatgaattcgcctacgagagtctgagaacacgaccagccgctccttaccaagtaccaaccataggggtgtatggcgtgccaggatcaggcaagtctggcatcattaaaagcgcagtcaccaaaaaagatctagtggtgagcgccaagaaagaaaactgtgcagaaattataagggacgtcaagaaaatgaaagggctggacgtcaatgccagaactgtggactcagtgctcttgaatggatgcaaacaccccgtagagaccctgtatattgacgaagcttttgcttgtcatgcaggtactctcagagcgctcatagccattataagacctaaaaaggcagtgctctgcggggatcccaaacagtgcggtttttttaacatgatgtgcctgaaagtgcattttaaccacgagatttgcacacaagtcttccacaaaagcatctctcgccgttgcactaaatctgtgacttcggtcgtctcaaccttgttttacgacaaaaaaatgagaacgacgaatccgaaagagactaagattgtgattgacactaccggcagtaccaaacctaagcaggacgatctcattctcacttgtttcagagggtgggtgaagcagttgcaaatagattacaaaggcaacgaaataatgacggcagctgcctctcaagggctgacccgtaaaggtgtgtatgccgttcggtacaaggtgaatgaaaatcctctgtacgcacccacctctgaacatgtgaacgtcctactgacccgcacggaggaccgcatcgtgtggaaaacactagccggcgacccatggataaaaacactgactgccaagtaccctgggaatttcactgccacgatagaggagtggcaagcagagcatgatgccatcatgaggcacatcttggagagaccggaccctaccgacgtcttccagaataaggcaaacgtgtgttgggccaaggctttagtgccggtgctgaagaccgctggcatagacatgaccactgaacaatggaacactgtggattattttgaaacggacaaagctcactcagcagagatagtattgaaccaactatgcgtgaggttctttggactcgatctggactccggtctattttctgcacccactgttccgttatccattaggaataatcactgggataactccccgtcgcctaacatgtacgggctgaataaagaagtggtccgtcagctctctcgcaggtacccacaactgcctcgggcagttgccactggaagagtctatgacatgaacactggtacactgcgcaattatgatccgcgcataaacctagtacctgtaaacagaagactgcctcatgctttagtcctccaccataatgaacacccacagagtgacttttcttcattcgtcagcaaattgaagggcagaactgtcctggtggtcggggaaaagttgtccgtcccaggcaaaatggttgactggttgtcagaccggcctgaggctaccttcagagctcggctggatttaggcatcccaggtgatgtgcccaaatatgacataatatttgttaatgtgaggaccccatataaataccatcactatcagcagtgtgaagaccatgccattaagcttagcatgttgaccaagaaagcttgtctgcatctgaatcccggcggaacctgtgtcagcataggttatggttacgctgacagggccagcgaaagcatcattggtgctatagcgcggcagttcaagttttcccgggtatgcaaaccgaaatcctcacttgaagagacggaagttctgtttgtattcattgggtacgatcgcaaggcccgtacgcacaatccttacaagctttcatcaaccttgaccaacatttatacaggttccagactccacgaagccggatgtgcaccctcatatcatgtggtgcgaggggatattgccacggccaccgaaggagtgattataaatgctgctaacagcaaaggacaacctggcggaggggtgtgcggagcgctgtataagaaattcccggaaagcttcgatttacagccgatcgaagtaggaaaagcgcgactggtcaaaggtgcagctaaacatatcattcatgccgtaggaccaaacttcaacaaagtttcggaggttgaaggtgacaaacagttggcagaggcttatgagtccatcgctaagattgtcaacgataacaattacaagtcagtagcgattccactgttgtccaccggcatcttttccgggaacaaagatcgactaacccaatcattgaaccatttgctgacagctttagacaccactgatgcagatgtagccatatactgcagggacaagaaatgggaaatgactctcaaggaagcagtggctaggagagaagcagtggaggagatatgcatatccgacgactcttcagtgacagaacctgatgcagagctggtgagggtgcatccgaagagttctttggctggaaggaagggctacagcacaagcgatggcaaaactttctcatatttggaagggaccaagtttcaccaggcggccaaggatatagcagaaattaatgccatgtggcccgttgcaacggaggccaatgagcaggtatgcatgtatatcctcggagaaagcatgagcagtattaggtcgaaatgccccgtcgaagagtcggaagcctccacaccacctagcacgctgccttgcttgtgcatccatgccatgactccagaaagagtacagcgcctaaaagcctcacgtccagaacaaattactgtgtgctcatcctttccattgccgaagtatagaatcactggtgtgcagaagatccaatgctcccagcctatattgttctcaccgaaagtgcctgcgtatattcatccaaggaagtatctcgtggaaacaccaccggtagacgagactccggagccatcggcagagaaccaatccacagaggggacacctgaacaaccaccacttataaccgaggatgagaccaggactagaacgcctgagccgatcatcatcgaagaggaagaagaggatagcataagtttgctgtcagatggcccgacccaccaggtgctgcaagtcgaggcagacattcacgggccgccctctgtatctagctcatcctggtccattcctcatgcatccgactttgatgtggacagtttatccatacttgacaccctggagggagctagcgtgaccagcggggcaacgtcagccgagactaactcttacttcgcaaagagtatggagtttctggcgcgaccggtgcctgcgcctcgaacagtattcaggaaccctccacatcccgctccgcgcacaagaacaccgtcacttgcacccagcagggcctgctcgagaaccagcctagtttccaccccgccaggcgtgaatagggtgatcactagagaggagctcgaggcgcttaccccgtcacgcactcctagcaggtcggtctcgagaaccagcctggtctccaacccgccaggcgtaaatagggtgattacaagagaggagtttgaggcgttcgtagcacaacaacaatgacggtttgatgcgggtgcatacatcttttcctccgacaccggtcaagggcatttacaacaaaaatcagtaaggcaaacggtgctatccgaagtggtgttggagaggaccgaattggagatttcgtatgccccgcgcctcgaccaagaaaaagaagaattactacgcaagaaattacagttaaatcccacacctgctaacagaagcagataccagtccaggaaggtggagaacatgaaagccataacagctagacgtattctgcaaggcctagggcattatttgaaggcagaaggaaaagtggagtgctaccgaaccctgcatcctgttcctttgtattcatctagtgtgaaccgtgccttttcaagccccaaggtcgcagtggaagcctgtaacgccatgttgaaagagaactttccgactgtggcttcttactgtattattccagagtacgatgcctatttggacatggttgacggagcttcatgctgcttagacactgccagtttttgccctgcaaagctgcgcagctttccaaagaaacactcctatttggaacccacaatacgatcggcagtgccttcagcgatccagaacacgctccagaacgtcctggcagctgccacaaaaagaaattgcaatgtcacgcaaatgagagaattgcccgtattggattcggcggcctttaatgtggaatgcttcaagaaatatgcgtgtaataatgaatattgggaaacgtttaaagaaaaccccatcaggcttactgaagaaaacgtggtaaattacattaccaaattaaaaggaccaaaagctgctgctctttttgcgaagacacataatttgaatatgttgcaggacataccaatggacaggtttgtaatggacttaaagagagacgtgaaagtgactccaggaacaaaacatactgaagaacggcccaaggtacaggtgatccaggctgccgatccgctagcaacagcgtatctgtgcggaatccaccgagagctggttaggagattaaatgcggtcctgcttccgaacattcatacactgtttgatatgtcggctgaagactttgacgctattatagccgagcacttccagcctggggattgtgttctggaaactgacatcgcgtcgtttgataaaagtgaggacgacgccatggctctgaccgcgttaatgattctggaagacttaggtgtggacgcagagctgttgacgctgattgaggcggctttcggcgaaatttcatcaatacatttgcccactaaaactaaatttaaattcggagccatgatgaaatctggaatgttcctcacactgtttgtgaacacagtcattaacattgtaatcgcaagcagagtgttgagagaacggctaaccggatcaccatgtgcagcattcattggagatgacaatatcgtgaaaggagtcaaatcggacaaattaatggcagacaggtgcgccacctggttgaatatggaagtcaagattatagatgctgtggtgggcgagaaagcgccttatttctgtggagggtttattttgtgtgactccgtgaccggcacagcgtgccgtgtggcagaccccctaaaaaggctgtttaagcttggcaaacctctggcagcagacgatgaacatgatgatgacaggagaagggcattgcatgaagagtcaacacgctggaaccgagtgggtattctttcagagctgtgcaaggcagtagaatcaaggtatgaaaccgtaggaacttccatcatagttatggccatgactactctagctagcagtgttaaatcattcagctacctgagaggggcccctataactctctacggctaacctgaatggactacgacatagtctagtccgccaagatatcgcaccatgggaagagccggcgtgagcaagggcgaggagctgttcaccggggtggtgcccatcctggtcgagctggacggcgacgtaaacggccacaagttcagcgtgtccggcgagggcgagggcgatgccacctacggcaagctgaccctgaagctgatctgcaccaccggcaagctgcccgtgccctggcccaccctcgtgaccaccctgggctacggcctgcagtgcttcgcccgctaccccgaccacatgaagcagcacgacttcttcaagtccgccatgcccgaaggctacgtccaggagcgcaccatcttcttcaaggacgacggcaactacaagacccgcgccgaggtgaagttcgagggcgacaccctggtgaaccgcatcgagctgaagggcatcgacttcaaggaggacggcaacatcctggggcacaagctggagtacaactacaacagccacaacgtctatatcaccgccgacaagcagaagaacggcatcaaggccaacttcaagatccgccacaacatcgaggacggcggcgtgcagctcgccgaccactaccagcagaacacccccatcggcgacggccccgtgctgctgcccgacaaccactacctgagctaccagtccgccctgagcaaagaccccaacgagaagcgcgatcacatggtcctgctggagttcgtgaccgccgccgggatcactctcggcatggacgagctgtacaagtaggctcttcgtaattaattgatcgatacagcagcaattggcaagctgcttacatagaaggcgcgccgtttaaacggccggccttaattaagtaacgatacagcagcaattggcaagctgcttacatagaactcgcggcgattggcatgccgctttaaaatttttattttatttttcttttcttttccgaatcggattttgtttttaatatttcaaaaaaaaaaaaaaaaaaaaaaaaaaaaaaaaaaaaaaaa

SEQ ID NO: 36 - DNA, 59 bp, Artificial Sequence
  Synthetic polynucleotide
  misc_feature: 5 human beta globin UTR
acatttgcttctgacacaactgtgttcactagcaacctcaaacagacaccgccgccacc

SEQ ID NO: 37 - DNA, 18 bp, Artificial Sequence
  Synthetic polynucleotide
  misc_feature: T7 Promoter
taatacgactcactatag

SEQ ID NO: 38 - DNA, 142 bp, Artificial Sequence
  Synthetic polynucleotide
  misc_feature: DLP
atagtcagcatagtacatttcatctgactaatactacaacaccaccaccatgaatagaggattctttaacatgctcggccgccgccccttcccggcccccactgccatgtggaggccgcggagaaggaggcaggcggccccg

SEQ ID NO: 39 - DNA, 66 bp, Artificial Sequence; identical to SEQ ID NO: 3
  Synthetic polynucleotide
  misc_feature: P2A

SEQ ID NO: 40 - DNA, 846 bp, Artificial Sequence
  Synthetic polynucleotide
  misc_feature: dsGFP
atggtgagcaagggcgaggagctgttcaccggggtggtgcccatcctggtcgagctggacggcgacgtaaacggccacaagttcagcgtgtccggcgagggcgagggcgatgccacctacggcaagctgaccctgaagttcatctgcaccaccggcaagctgcccgtgccctggcccaccctcgtgaccaccctgacctacggcgtgcagtgcttcagccgctaccccgaccacatgaagcagcacgacttcttcaagtccgccatgcccgaaggctacgtccaggagcgcaccatcttcttcaaggacgacggcaactacaagacccgcgccgaggtgaagttcgagggcgacaccctggtgaaccgcatcgagctgaagggcatcgacttcaaggaggacggcaacatcctggggcacaagctggagtacaactacaacagccacaacgtctatatcatggccgacaagcagaagaacggcatcaaggtgaacttcaagatccgccacaacatcgaggacggcagcgtgcagctcgccgaccactaccagcagaacacccccatcggcgacggccccgtgctgctgcccgacaaccactacctgagcacccagtccgccctgagcaaagaccccaacgagaagcgcgatcacatggtcctgctggagttcgtgaccgccgccgggatcactctcggcatggacgagctgtacaagaagcttagccatggcttcccgccggaggtggaggagcaggatgatggcacgctgcccatgtcttgtgcccaggagagcgggatggaccgtcaccctgcagcctgtgcttctgctaggatcaatgtgtag

SEQ ID NO: 41 - DNA, 134 bp, Artificial Sequence
  Synthetic polynucleotide
  misc_feature: 3 Human beta globin UTR
gctcgctttcttgctgtccaatttctattaaaggttcctttgttccctaagtccaactactaaactgggggatattatgaagggccttgagcatctggattctgcctaataaaaaacatttattttcattgcaa

SEQ ID NO: 42 - DNA, 29 bp, Artificial Sequence
  Synthetic polynucleotide
  misc_feature: T7 Terminator
aacccctctctaaacggaggggttttttt

SEQ ID NO: 43 - DNA, 1412 bp, Artificial Sequence
  Synthetic polynucleotide
  misc_feature: Sequence of DLP dsGFP Mrna
taatacgactcactatagacatttgcttctgacacaactgtgttcactagcaacctcaaacagacaccgccgccaccatagtcagcatagtacatttcatctgactaatactacaacaccaccaccatgaatagaggattctttaacatgctcggccgccgccccttcccggcccccactgccatgtggaggccgcggagaaggaggcaggcggccccgggaagcggagctactaacttcagcctgctgaagcaggctggagacgtggaggagaaccctggacctatggtgagcaagggcgaggagctgttcaccggggtggtgcccatcctggtcgagctggacggcgacgtaaacggccacaagttcagcgtgtccggcgagggcgagggcgatgccacctacggcaagctgaccctgaagttcatctgcaccaccggcaagctgcccgtgccctggcccaccctcgtgaccaccctgacctacggcgtgcagtgcttcagccgctaccccgaccacatgaagcagcacgacttcttcaagtccgccatgcccgaaggctacgtccaggagcgcaccatcttcttcaaggacgacggcaactacaagacccgcgccgaggtgaagttcgagggcgacaccctggtgaaccgcatcgagctgaagggcatcgacttcaaggaggacggcaacatcctggggcacaagctggagtacaactacaacagccacaacgtctatatcatggccgacaagcagaagaacggcatcaaggtgaacttcaagatccgccacaacatcgaggacggcagcgtgcagctcgccgaccactaccagcagaacacccccatcggcgacggccccgtgctgctgcccgacaaccactacctgagcacccagtccgccctgagcaaagaccccaacgagaagcgcgatcacatggtcctgctggagttcgtgaccgccgccgggatcactctcggcatggacgagctgtacaagaagcttagccatggcttcccgccggaggtggaggagcaggatgatggcacgctgcccatgtcttgtgcccaggagagcgggatggaccgtcaccctgcagcctgtgcttctgctaggatcaatgtgtaggctcgctttcttgctgtccaatttctattaaaggttcctttgttccctaagtccaactactaaactgggggatattatgaagggccttgagcatctggattctgcctaataaaaaacatttattttcattgcaaaaaaaaaaaaaaaaaaaaaaaaaaaaaaaaaaaaaaaaaaaaaaaaaaaaaaaaaaaaaaaaaaaaaaaaaaaaaaaaaaaaaaaaaaaaaaaaaaaaaaaaaaaaaaaaaaaaaaaaaacccctctctaaacggaggggttttttt

SEQ ID NO: 44 - protein, 9 aa, Artificial Sequence
  Synthetic polypeptide
  misc_feature: H-2 Kd peptide
IYSTVASSL

SEQ ID NO: 45 - protein, 15 aa, Artificial Sequence
  Synthetic polypeptide
  misc_feature: CD4 T cell epitope
KSSFFRNVVWLIKKN

SEQ ID NO: 46 - DNA, 104 bp, Sindbis virus
atgaatagaggattctttaacatgctcggccgccgccccttcccggcccccactgccatgtggaggccgcggagaaggaggcaggcggccccgatgcctgcccg

SEQ ID NO: 47 - DNA, 120 bp, Aura virus
atgaactctgtcttttacaatccgtttggccgaggtgcctacgctcaacctccaatagcatggaggccaagacgtagggctgcacctgcgcctcgaccatccgggttgactacccagatc

SEQ ID NO: 48 - DNA, 71 bp, Eastern Equine Encephalitis virus SA
atgtttccgtatccaacattgaactacccgcctatggcaccggttaatccgatggcatacagggaccccaa

SEQ ID NO: 49 - DNA, 91 bp, O'Nyong-Nyong virus
atggagttcataccagcacaaacttactacaatagaagataccagcctagaccctggactcaacgccctactatccaggtgatcaggccaa

SEQ ID NO: 50 - DNA, 67 bp, Semliki Forest virus
atgaattacatccctacgcaaacgttttacggccgccggtggcgcccgcgcccggcggcccgtcctt

SEQ ID NO: 51 - DNA, 69 bp, Ross River virus
atgaattacataccaacccagactttttacggacgccgttggcggcctcgcccggcgttccgtccatgg

SEQ ID NO: 52 - DNA, 91 bp, Mayaro virus
atggatttcctaccaacacaagtgttttatggcaggcgatggagaccacgaatgccgccacgcccttggaggccacgcccacctacaattc